European Patent Application EP 4 721 728 A1, published April 8, 2026. Title: 一种低空载率的核酸脂质纳米颗粒及其制备方法. Applicant: 石药集团中奇制药技术（石家庄）有限公司. The sequence listing filed with the application follows.

SEQUENCE LISTING (32 sequences)

SEQ ID NO: 1 - RNA, 4360 nt, synthetic construct
  source 1..4360: mol_type = other RNA
gggagacccaagctggctagcgtttaaacttaagcttggtaccgagctcggatccactagtccagtgtggtggaattcgaataaactagtattcttctggtccccacagactcagagagaacccgccaccatgttcgtgttcctggtgctgctgcccttagtgagcagccagtgcgtcaacctaactactagaacacagctgcctcctgcctacacaaacagcttcaccagaggcgtgtattaccccgataaggtgttccggtcttctgtgctgcacagcacccaggacctgtttctgcctttcttcagcaatgtgacctggttccacgccatccacgtgtctggcacaaacggcacaaaaaggttcgacaaccccgttctgcctttcaatgacggcgtgtacttcgctagcacagaaaagagcaacatcatcagaggatggatcttcggaaccaccctggattccaagacacagtccctgttgatcgttaataatgccaccaatgtggtgatcaaggtgtgtgagttccagttttgcaacgatccttttctgggcgtgtattaccacaagaataacaaaagctggatggaaagcgagtttagagtatactctagcgccaacaactgcaccttcgagtacgtcagccagccttttctgatggacctggaaggcaagcagggcaacttcaagaatctgagagagttcgtgttcaaaaacattgacggatatttcaaaatctacagcaagcacacacctatcaatctggtgcgggacctgccacaggggtttagcgcattggagcctctggtcgatctgcctatcggcatcaacatcacccggttccagaccctgctagccctgcatagaagctatctgacccctggcgacagctcaagcggctggaccgccggcgccgccgcctactacgtgggctacctgcagcctagaacctttctgctgaagtacaacgagaacggcaccataaccgacgctgtggactgcgccctggaccccctgtctgaaaccaagtgcaccctgaagagctttaccgtggaaaagggcatctaccaaacaagcaatttccgggtgcagcctaccgagtctatcgtgcggtttcccaacatcaccaacctgtgcccattcggagaagtgttcaacgccaccagattcgccagcgtgtacgcctggaaccggaagagaatctctaactgcgtggccgattacagcgtgctctataactcggctagcttcagcacattcaagtgctacggcgtgagccccacaaagctgaacgacctgtgcttcaccaacgtctacgccgacagcttcgtgattagaggcgatgaggtccgacagatcgcccctggccaaaccggcaagattgctgactacaactacaagctgcctgatgacttcactggatgtgtgatcgcttggaactccaacaacctggactctaaagtgggcggaaactacaactaccggtaccggctgtttagaaagagtaaccttaaacctttcgagagagatatcagcacagaaatctaccaggctggcagcacaccttgtaacggcgtgcaaggcttcaactgctatttccctctccagtcttatggcttccagcctaccaacggcgtgggctatcagccctaccgagtggtggtgctgtccttcgagctgctgcatgcccctgctaccgtgtgcggccctaagaaatcgaccaacctggtgaagaacaagtgcgtgaattttaatttcaacggcctcaccggcaccggagtgctgaccgagagcaacaagaagttcctgcccttccagcagttcggaagagacatcgccgataccacagacgccgtgcgggacccccaaacactggaaatcctggacatcacaccttgcagcttcggcggcgtgagcgtgatcacccctggcaccaacacaagcaaccaggtggccgtgctctaccagggcgtgaactgcaccgaagtgccagtggccatccacgccgatcagctgacccctacctggagagtgtacagcaccggcagcaacgtgttccagacaagggctggttgtctgatcggcgccgagcacgtgaataattcctacgagtgcgacatccctattggcgccggaatctgtgccagctaccagacacagacaaactccccacgtagagccagatccgtcgccagccagagcatcatcgcttacaccatgagcctgggcgctgaaaacagcgtggcttacagcaacaattctatcgccatacctaccaattttacaatctcggtgacaaccgagatcctgcctgttagcatgaccaagaccagcgtggactgcacaatgtacatctgcggagacagcaccgagtgctccaacctgctgcttcaatacgggtccttctgtacacagctgaatagagccctgacaggcatcgctgttgagcaggacaagaacacccaggaggtgtttgcccaagtgaagcagatctacaagactccgcctatcaaggacttcggcggcttcaacttcagccagatcctgccagatccttctaagcctagcaagcgcagtttcatcgaggacctgttgttcaacaaggtgaccctggccgacgccggctttatcaagcagtacggcgattgcctgggcgacatcgccgctagagatctgatctgcgcccagaagttcaatggactgacagtgctgccgcccctgctgaccgatgagatgatcgctcagtacacctctgccctgctggccgggacaatcaccagcggatggacattcggggccggcgccgccctgcagatcccctttgccatgcagatggcctacagattcaacggtattggcgtgacccaaaacgtgctgtacgagaatcagaagttaatcgcaaaccagttcaacagcgccatcggcaagatccaggattccctgagttccacggccagcgctctgggtaagctgcaagacgtggtgaaccagaacgcacaggccctgaacaccctggtcaaacagctgagctccaacttcggagcgatcagcagcgtgcttaatgacatcctgagcagactggatccccccgaggccgaagtccaaatcgaccggctgatcacaggcaggttgcagagcctgcagacctacgtgacccaacagctgatcagagcagccgagatcagagcctcagccaatctggctgctacgaagatgagcgagtgtgtgctgggacagagcaagcgggtggatttttgcggcaaagggtaccacctgatgagcttccctcagagcgcccctcacggcgttgtgttcctgcacgtgacgtacgtgcccgcccaagagaagaacttcaccacagcccctgccatctgccacgacggaaaagcccacttccctcgtgagggcgtcttcgtgagcaacggcacacactggttcgtgactcagagaaacttctacgagcctcagatcatcaccaccgacaacacctttgtgagcggcaactgcgacgtggtgatcgggatcgtgaacaacaccgtgtacgaccccctgcagcctgagctggatagcttcaaagaggaactggacaagtatttcaagaatcacacctctccagacgtggacctgggcgacatcagcggcattaacgcctctgtggtgaacatccagaaggaaatcgatcggctgaacgaggtggccaagaacttgaacgagagcctgatcgacctgcaggagctgggcaagtacgagcagtacatcaagtggccttggtacatctggctgggattcatcgccggcctgattgccatcgtcatggtgaccatcatgctgtgttgcatgacaagctgctgcagctgtctgaagggatgttgctcttgtggctcttgctgtaaattcgacgaagacgactcggaacccgtgctgaagggcgttaagctccactacacctgatgactcgagctggtactgcatgcacgcaatgctagctgcccctttcccgtcctgggtaccccgagtctcccccgacctcgggtcccaggtatgctcccacctccacctgccccactcaccacctctgctagttccagacacctcccaagcacgcagcaatgcagctcaaaacgcttagcctagccacacccccacgggaaacagcagtgattaacctttagcaataaacgaaagtttaactaagctatactaaccccagggttggtcaatttcgtgccagccacaccctggagctagcaaaaaaaaaaaaaaaaaaaaaaaaaaaaaagcatatgactaaaaaaaaaaaaaaaaaaaaaaaaaaaaaaaaaaaaaaaaaaaaaaaaaaaaaaaaaaaaaaaaaaaaaa

SEQ ID NO: 2 - RNA, 4360 nt, synthetic construct
  source 1..4360: mol_type = other RNA
gggagacccaagctggctagcgtttaaacttaagcttggtaccgagctcggatccactagtccagtgtggtggaattcgaataaactagtattcttctggtccccacagactcagagagaacccgccaccatgttcgtgttcctggtcctgctgcccctggtgtctagtcagtgtgtgaacctgacaacccgcacccagctgccccctgcctacactaactcttttaccaggggagtgtactacccagacaaagtgtttagatcttctgtgctgcactctacacaggatctgtttctgccattcttctctaacgtgacatggttccacgccattcacgtcagtggaactaacggcactaagagattcgacaaccccgtgctgcctttcaacgacggagtgtacttcgcgagcactgagaagtccaacatcatcagaggctggatctttggcaccacactggatagcaagacacagagtctgctgattgtgaacaacgccactaatgttgtgatcaaggtgtgtgagttccagttctgcaacgatccttttctgggggtgtattaccacaaaaacaacaagagttggatggagtcagagtttagggtgtattcttccgcaaacaactgtacattcgaatacgtctcccagccatttctgatggacctggaggggaagcagggcaactttaaaaatctgcgcgagtttgtgttcaagaacatcgatgggtactttaagatttactccaaacacacacctatcaacctggtgagagatctgccacagggattcagcgccctggagccactggtggatctgccaatcggaatcaatatcacaagattccagacattactcgctctgcacaggtcctatctgactccaggtgatagcagcagcggttggactgctggagcagctgcctactatgtgggatacctgcagccaagaacattcctgttgaaatacaacgagaatggaacaatcacagatgctgtggactgtgcactggatccactgtctgagaccaagtgcacactgaagagcttcactgtcgagaagggcatctatcagacatctaactttagagtgcagcccacagagagcatcgtgcgattccccaacatcacaaacctgtgtccttttggcgaggtgttcaacgccacaagattcgcttctgtgtacgcatggaacaggaagcgaatctctaactgtgtggccgattacagcgtgctgtacaactctgcttctttctccacattcaagtgttacggagtgtcacctactaaactgaacgacctgtgcttcactaacgtgtatgccgatagtttcgtgatccggggagatgaggtgaggcagatcgccccaggacagaccgggaaaatcgccgattacaactataagctgccagacgatttcaccggttgtgtgatcgcctggaactcaaacaacctggatagcaaagtggggggcaactataactacagataccgactgttcaggaaaagcaacctgaaaccttttgagcgcgatatctccactgagatctaccaggcaggatctacaccatgtaatggagtgcagggattcaactgttacttccccctccagtcttatggctttcagcctactaacggagtgggatatcagccctacagagtggtggtcctgtccttcgagctgctgcacgcacccgctaccgtgtgcggacctaagaagtcaaccaacctggtgaaaaacaagtgtgtaaactttaacttcaacggactcaccggcaccggagttctgacagagtctaacaaaaagttcctgcccttccagcagttcggcagggatatcgctgacaccactgacgctgtgagagacccacagaccctggagatcctggatatcaccccttgttctttcggcggtgtcagtgtgatcacaccaggaactaacaccagtaaccaggtggccgtgctctaccagggagtgaactgtaccgaggtgcctgtggctatccacgccgaccagctgacccctacctggagggtgtatagcaccggatctaacgtgttccagacacgagccggctgcctcatcggcgccgagcacgtgaacaactcttacgagtgtgacatccctatcggagctggaatctgtgcttcctaccagacacagaccaattctcctagaagagccagatctgtcgcaagccagagtatcatcgcttacaccatgagcctgggagctgagaacagcgtggcttacagcaacaacagcatcgcaatccctaccaatttcacaatctcagtgactaccgagatcctgcccgtgagcatgactaaaacatcagtggactgtacaatgtatatctgcggagactccacagagtgctcaaacctgctgctgcagtatggatctttctgtactcagctgaacagagctctgacaggaatcgcagtggagcaggacaagaacactcaggaggtgtttgcccaggtgaagcagatctacaaaacccctcctatcaaagattttgggggattcaacttcagccagatcctgcctgatccttccaaaccttccaaaagatcatttatcgaggaccttctgttcaacaaggtcaccctggctgacgctggctttatcaagcagtatggcgattgtctgggtgatatcgcagcaagagatctgatttgtgctcagaagtttaacggactgacagttctgcctccgctgctgaccgatgagatgatcgcccagtacacaagtgcactgctggctggcaccatcacatccggctggaccttcggagccggcgccgccctgcagattcctttcgctatgcagatggcatatcgctttaacggaattggcgtgactcagaacgtcctgtacgagaaccagaaactgatcgcaaaccagttcaacagcgctatcggaaaaatccaggatagcctgtcatctacagccagtgccctgggaaagctgcaggacgtggtgaatcagaacgcacaggccctgaacacactggtgaaacagctgagctcaaactttggagctatctcctcggtcctgaacgacatcctgtccagactggatccgcctgaggctgaggtgcagatcgacagactgatcacaggaagactgcagagtctgcaaacctacgtgacccagcagctcatccgcgctgctgagatcagagcgtccgcaaacctggcagccaccaaaatgagtgagtgtgtgctcggacagagcaaacgcgtggatttctgtggcaagggataccatctgatgagcttcccacagagcgccccacacggagtggtgttcctgcatgtgacttacgtccccgctcaggagaaaaatttcacaactgcgcctgctatctgccacgatggtaaggctcactttccaagagagggagtgtttgtgagcaatgggacacattggttcgtcacccagagaaacttctacgagcctcagatcatcactaccgacaatactttcgtgtcaggaaactgcgacgtggtgatcggcatcgtcaacaataccgtttacgaccctctgcagcctgagctggacagtttcaaagaggagctggataaatacttcaaaaaccacactagcccagacgtggacctgggagatatcagcggcatcaatgcatctgtggtgaacatccagaaagagattgacagactgaacgaggtggccaagaacctgaacgaaagtctgatcgatctgcaagagctgggaaaatatgagcagtacatcaaatggccttggtacatttggctgggattcatcgctggactgatcgcaattgtgatggtgacaattatgctgtgctgcatgacaagctgctgttcttgtctcaaaggatgctgctcttgcggtagctgctgtaaatttgatgaggacgatagtgagcctgtgctcaagggagtcaaactgcactatacctaatgactcgagctggtactgcatgcacgcaatgctagctgcccctttcccgtcctgggtaccccgagtctcccccgacctcgggtcccaggtatgctcccacctccacctgccccactcaccacctctgctagttccagacacctcccaagcacgcagcaatgcagctcaaaacgcttagcctagccacacccccacgggaaacagcagtgattaacctttagcaataaacgaaagtttaactaagctatactaaccccagggttggtcaatttcgtgccagccacaccctggagctagcaaaaaaaaaaaaaaaaaaaaaaaaaaaaaagcatatgactaaaaaaaaaaaaaaaaaaaaaaaaaaaaaaaaaaaaaaaaaaaaaaaaaaaaaaaaaaaaaaaaaaaaaa

SEQ ID NO: 3 - RNA, 4692 nt, synthetic construct
  source 1..4692: mol_type = other RNA
gggagacccaagctggctagcgtttaaacttaagcttggtaccgagctcggatccactagtccagtgtggtggaattcgaataaactagtattcttctggtccccacagactcagagagaacccgccaccatgttcgtgttcctggtgctgctgcccttagtgagcagccagtgcgtcaacctaactactagaacacagctgcctcctgcctacacaaacagcttcaccagaggcgtgtattaccccgataaggtgttccggtcttctgtgctgcacagcacccaggacctgtttctgcctttcttcagcaatgtgacctggttccacgccatccacgtgtctggcacaaacggcacaaaaaggttcgacaaccccgttctgcctttcaatgacggcgtgtacttcgctagcacagaaaagagcaacatcatcagaggatggatcttcggaaccaccctggattccaagacacagtccctgttgatcgttaataatgccaccaatgtggtgatcaaggtgtgtgagttccagttttgcaacgatccttttctgggcgtgtattaccacaagaataacaaaagctggatggaaagcgagtttagagtatactctagcgccaacaactgcaccttcgagtacgtcagccagccttttctgatggacctggaaggcaagcagggcaacttcaagaatctgagagagttcgtgttcaaaaacattgacggatatttcaaaatctacagcaagcacacacctatcaatctggtgcgggacctgccacaggggtttagcgcattggagcctctggtcgatctgcctatcggcatcaacatcacccggttccagaccctgctagccctgcatagaagctatctgacccctggcgacagctcaagcggctggaccgccggcgccgccgcctactacgtgggctacctgcagcctagaacctttctgctgaagtacaacgagaacggcaccataaccgacgctgtggactgcgccctggaccccctgtctgaaaccaagtgcaccctgaagagctttaccgtggaaaagggcatctaccaaacaagcaatttccgggtgcagcctaccgagtctatcgtgcggtttcccaacatcaccaacctgtgcccattcggagaagtgttcaacgccaccagattcgccagcgtgtacgcctggaaccggaagagaatctctaactgcgtggccgattacagcgtgctctataactcggctagcttcagcacattcaagtgctacggcgtgagccccacaaagctgaacgacctgtgcttcaccaacgtctacgccgacagcttcgtgattagaggcgatgaggtccgacagatcgcccctggccaaaccggcaagattgctgactacaactacaagctgcctgatgacttcactggatgtgtgatcgcttggaactccaacaacctggactctaaagtgggcggaaactacaactaccggtaccggctgtttagaaagagtaaccttaaacctttcgagagagatatcagcacagaaatctaccaggctggcagcacaccttgtaacggcgtgcaaggcttcaactgctatttccctctccagtcttatggcttccagcctaccaacggcgtgggctatcagccctaccgagtggtggtgctgtccttcgagctgctgcatgcccctgctaccgtgtgcggccctaagaaatcgaccaacctggtgaagaacaagtgcgtgaattttaatttcaacggcctcaccggcaccggagtgctgaccgagagcaacaagaagttcctgcccttccagcagttcggaagagacatcgccgataccacagacgccgtgcgggacccccaaacactggaaatcctggacatcacaccttgcagcttcggcggcgtgagcgtgatcacccctggcaccaacacaagcaaccaggtggccgtgctctaccagggcgtgaactgcaccgaagtgccagtggccatccacgccgatcagctgacccctacctggagagtgtacagcaccggcagcaacgtgttccagacaagggctggttgtctgatcggcgccgagcacgtgaataattcctacgagtgcgacatccctattggcgccggaatctgtgccagctaccagacacagacaaactccccacgtagagccagatccgtcgccagccagagcatcatcgcttacaccatgagcctgggcgctgaaaacagcgtggcttacagcaacaattctatcgccatacctaccaattttacaatctcggtgacaaccgagatcctgcctgttagcatgaccaagaccagcgtggactgcacaatgtacatctgcggagacagcaccgagtgctccaacctgctgcttcaatacgggtccttctgtacacagctgaatagagccctgacaggcatcgctgttgagcaggacaagaacacccaggaggtgtttgcccaagtgaagcagatctacaagactccgcctatcaaggacttcggcggcttcaacttcagccagatcctgccagatccttctaagcctagcaagcgcagtttcatcgaggacctgttgttcaacaaggtgaccctggccgacgccggctttatcaagcagtacggcgattgcctgggcgacatcgccgctagagatctgatctgcgcccagaagttcaatggactgacagtgctgccgcccctgctgaccgatgagatgatcgctcagtacacctctgccctgctggccgggacaatcaccagcggatggacattcggggccggcgccgccctgcagatcccctttgccatgcagatggcctacagattcaacggtattggcgtgacccaaaacgtgctgtacgagaatcagaagttaatcgcaaaccagttcaacagcgccatcggcaagatccaggattccctgagttccacggccagcgctctgggtaagctgcaagacgtggtgaaccagaacgcacaggccctgaacaccctggtcaaacagctgagctccaacttcggagcgatcagcagcgtgcttaatgacatcctgagcagactggatccccccgaggccgaagtccaaatcgaccggctgatcacaggcaggttgcagagcctgcagacctacgtgacccaacagctgatcagagcagccgagatcagagcctcagccaatctggctgctacgaagatgagcgagtgtgtgctgggacagagcaagcgggtggatttttgcggcaaagggtaccacctgatgagcttccctcagagcgcccctcacggcgttgtgttcctgcacgtgacgtacgtgcccgcccaagagaagaacttcaccacagcccctgccatctgccacgacggaaaagcccacttccctcgtgagggcgtcttcgtgagcaacggcacacactggttcgtgactcagagaaacttctacgagcctcagatcatcaccaccgacaacacctttgtgagcggcaactgcgacgtggtgatcgggatcgtgaacaacaccgtgtacgaccccctgcagcctgagctggatagcttcaaagaggaactggacaagtatttcaagaatcacacctctccagacgtggacctgggcgacatcagcggcattaacgcctctgtggtgaacatccagaaggaaatcgatcggctgaacgaggtggccaagaacttgaacgagagcctgatcgacctgcaggagctgggcaagtacgagcagtacatcaagtggccttggtacatctggctgggattcatcgccggcctgattgccatcgtcatggtgaccatcatgctgtgttgcatgacaagctgctgcagctgtctgaagggatgttgctcttgtggctcttgctgtaaattcgacgaagacgactcggaacccgtgctgaagggcgttaagctccactacacctgatgacaagcacgcagcaatgcagctcaaaacgcttagcctagccacacccccacgggaaacagcagtgattaacctttagcaataaacgaaagtttaactaagctatactaaccccagggttggtcaatttcgtgccagccacctcgagctggtactgcatgcacgcaatgctagctgcccctttcccgtcctgggtaccccgagtctcccccgacctcgggtcccaggtatgctcccacctccacctgccccactcaccacctctgctagttccagacacctccgctcgctttcttgctgtccaatttctattaaaggttcctttgttccctaagtccaactactaaactgggggatattatgaagggccttgagcatctggattctgcctaataaaaaacatttattttcattgcaattgccatgtgtatgtgggttcgcccacatactctgatgatccccaatcgtggcgtgtcggcctgcttcggcaggcactggcgccgggatcattcatggcaagctggagcctcggtggccatgcttcttgccccttgggcctccccccagcccctcctccccttcctgcacccgtacccccgtggtctttgaataaagtctgagtgggcggcaaaaaaaaaaaaaaaaaaaaaaaaaaaaaaagcatatgactaaaaaaaaaaaaaaaaaaaaaaaaaaaaaaaaaaaaaaaaaaaaaaaaaaaaaaaaaaaaaaaaaaaaaa

SEQ ID NO: 4 - RNA, 4553 nt, synthetic construct
  source 1..4553: mol_type = other RNA
gggagacccaagctggctagcgtttaaacttaagcttggtaccgagctcggatccactagtccagtgtggtggaattcgaataaactagtattcttctggtccccacagactcagagagaacccgccaccatgttcgtgttcctggtgctgctgcccttagtgagcagccagtgcgtcaacctaactactagaacacagctgcctcctgcctacacaaacagcttcaccagaggcgtgtattaccccgataaggtgttccggtcttctgtgctgcacagcacccaggacctgtttctgcctttcttcagcaatgtgacctggttccacgccatccacgtgtctggcacaaacggcacaaaaaggttcgacaaccccgttctgcctttcaatgacggcgtgtacttcgctagcacagaaaagagcaacatcatcagaggatggatcttcggaaccaccctggattccaagacacagtccctgttgatcgttaataatgccaccaatgtggtgatcaaggtgtgtgagttccagttttgcaacgatccttttctgggcgtgtattaccacaagaataacaaaagctggatggaaagcgagtttagagtatactctagcgccaacaactgcaccttcgagtacgtcagccagccttttctgatggacctggaaggcaagcagggcaacttcaagaatctgagagagttcgtgttcaaaaacattgacggatatttcaaaatctacagcaagcacacacctatcaatctggtgcgggacctgccacaggggtttagcgcattggagcctctggtcgatctgcctatcggcatcaacatcacccggttccagaccctgctagccctgcatagaagctatctgacccctggcgacagctcaagcggctggaccgccggcgccgccgcctactacgtgggctacctgcagcctagaacctttctgctgaagtacaacgagaacggcaccataaccgacgctgtggactgcgccctggaccccctgtctgaaaccaagtgcaccctgaagagctttaccgtggaaaagggcatctaccaaacaagcaatttccgggtgcagcctaccgagtctatcgtgcggtttcccaacatcaccaacctgtgcccattcggagaagtgttcaacgccaccagattcgccagcgtgtacgcctggaaccggaagagaatctctaactgcgtggccgattacagcgtgctctataactcggctagcttcagcacattcaagtgctacggcgtgagccccacaaagctgaacgacctgtgcttcaccaacgtctacgccgacagcttcgtgattagaggcgatgaggtccgacagatcgcccctggccaaaccggcaagattgctgactacaactacaagctgcctgatgacttcactggatgtgtgatcgcttggaactccaacaacctggactctaaagtgggcggaaactacaactaccggtaccggctgtttagaaagagtaaccttaaacctttcgagagagatatcagcacagaaatctaccaggctggcagcacaccttgtaacggcgtgcaaggcttcaactgctatttccctctccagtcttatggcttccagcctaccaacggcgtgggctatcagccctaccgagtggtggtgctgtccttcgagctgctgcatgcccctgctaccgtgtgcggccctaagaaatcgaccaacctggtgaagaacaagtgcgtgaattttaatttcaacggcctcaccggcaccggagtgctgaccgagagcaacaagaagttcctgcccttccagcagttcggaagagacatcgccgataccacagacgccgtgcgggacccccaaacactggaaatcctggacatcacaccttgcagcttcggcggcgtgagcgtgatcacccctggcaccaacacaagcaaccaggtggccgtgctctaccagggcgtgaactgcaccgaagtgccagtggccatccacgccgatcagctgacccctacctggagagtgtacagcaccggcagcaacgtgttccagacaagggctggttgtctgatcggcgccgagcacgtgaataattcctacgagtgcgacatccctattggcgccggaatctgtgccagctaccagacacagacaaactccccacgtagagccagatccgtcgccagccagagcatcatcgcttacaccatgagcctgggcgctgaaaacagcgtggcttacagcaacaattctatcgccatacctaccaattttacaatctcggtgacaaccgagatcctgcctgttagcatgaccaagaccagcgtggactgcacaatgtacatctgcggagacagcaccgagtgctccaacctgctgcttcaatacgggtccttctgtacacagctgaatagagccctgacaggcatcgctgttgagcaggacaagaacacccaggaggtgtttgcccaagtgaagcagatctacaagactccgcctatcaaggacttcggcggcttcaacttcagccagatcctgccagatccttctaagcctagcaagcgcagtttcatcgaggacctgttgttcaacaaggtgaccctggccgacgccggctttatcaagcagtacggcgattgcctgggcgacatcgccgctagagatctgatctgcgcccagaagttcaatggactgacagtgctgccgcccctgctgaccgatgagatgatcgctcagtacacctctgccctgctggccgggacaatcaccagcggatggacattcggggccggcgccgccctgcagatcccctttgccatgcagatggcctacagattcaacggtattggcgtgacccaaaacgtgctgtacgagaatcagaagttaatcgcaaaccagttcaacagcgccatcggcaagatccaggattccctgagttccacggccagcgctctgggtaagctgcaagacgtggtgaaccagaacgcacaggccctgaacaccctggtcaaacagctgagctccaacttcggagcgatcagcagcgtgcttaatgacatcctgagcagactggatccccccgaggccgaagtccaaatcgaccggctgatcacaggcaggttgcagagcctgcagacctacgtgacccaacagctgatcagagcagccgagatcagagcctcagccaatctggctgctacgaagatgagcgagtgtgtgctgggacagagcaagcgggtggatttttgcggcaaagggtaccacctgatgagcttccctcagagcgcccctcacggcgttgtgttcctgcacgtgacgtacgtgcccgcccaagagaagaacttcaccacagcccctgccatctgccacgacggaaaagcccacttccctcgtgagggcgtcttcgtgagcaacggcacacactggttcgtgactcagagaaacttctacgagcctcagatcatcaccaccgacaacacctttgtgagcggcaactgcgacgtggtgatcgggatcgtgaacaacaccgtgtacgaccccctgcagcctgagctggatagcttcaaagaggaactggacaagtatttcaagaatcacacctctccagacgtggacctgggcgacatcagcggcattaacgcctctgtggtgaacatccagaaggaaatcgatcggctgaacgaggtggccaagaacttgaacgagagcctgatcgacctgcaggagctgggcaagtacgagcagtacatcaagtggccttggtacatctggctgggattcatcgccggcctgattgccatcgtcatggtgaccatcatgctgtgttgcatgacaagctgctgcagctgtctgaagggatgttgctcttgtggctcttgctgtaaattcgacgaagacgactcggaacccgtgctgaagggcgttaagctccactacacctgatgagctcgctttcttgctgtccaatttctattaaaggttcctttgttccctaagtccaactactaaactgggggatattatgaagggccttgagcatctggattctgcctaataaaaaacatttattttcattgcaattgccatgtgtatgtgggttcgcccacatactctgatgatccccaatcgtggcgtgtcggcctgcttcggcaggcactggcgccgggatcattcatggcaagctggagcctcggtggccatgcttcttgccccttgggcctccccccagcccctcctccccttcctgcacccgtacccccgtggtctttgaataaagtctgagtgggcggcactcgagctggtactgcatgcacgcaatgctagctgcccctttcccgtcctgggtaccccgagtctcccccgacctcgggtcccaggtatgctcccacctccacctgccccactcaccacctctgctagttccagacacctccaaaaaaaaaaaaaaaaaaaaaaaaaaaaaagcatatgactaaaaaaaaaaaaaaaaaaaaaaaaaaaaaaaaaaaaaaaaaaaaaaaaaaaaaaaaaaaaaaaaaaaaaa

SEQ ID NO: 5 - RNA, 4332 nt, synthetic construct
  source 1..4332: mol_type = other RNA
gggagacccaagctggctagcgtttaaacttaagcttggtaccgagctcggatccactagtccagtgtggtggaattcgaataaactagtattcttctggtccccacagactcagagagaacccgccaccatgttcgtgttcctggtgctgctgcccttagtgagcagccagtgcgtcaacctaactactagaacacagctgcctcctgcctacacaaacagcttcaccagaggcgtgtattaccccgataaggtgttccggtcttctgtgctgcacagcacccaggacctgtttctgcctttcttcagcaatgtgacctggttccacgccatccacgtgtctggcacaaacggcacaaaaaggttcgacaaccccgttctgcctttcaatgacggcgtgtacttcgctagcacagaaaagagcaacatcatcagaggatggatcttcggaaccaccctggattccaagacacagtccctgttgatcgttaataatgccaccaatgtggtgatcaaggtgtgtgagttccagttttgcaacgatccttttctgggcgtgtattaccacaagaataacaaaagctggatggaaagcgagtttagagtatactctagcgccaacaactgcaccttcgagtacgtcagccagccttttctgatggacctggaaggcaagcagggcaacttcaagaatctgagagagttcgtgttcaaaaacattgacggatatttcaaaatctacagcaagcacacacctatcaatctggtgcgggacctgccacaggggtttagcgcattggagcctctggtcgatctgcctatcggcatcaacatcacccggttccagaccctgctagccctgcatagaagctatctgacccctggcgacagctcaagcggctggaccgccggcgccgccgcctactacgtgggctacctgcagcctagaacctttctgctgaagtacaacgagaacggcaccataaccgacgctgtggactgcgccctggaccccctgtctgaaaccaagtgcaccctgaagagctttaccgtggaaaagggcatctaccaaacaagcaatttccgggtgcagcctaccgagtctatcgtgcggtttcccaacatcaccaacctgtgcccattcggagaagtgttcaacgccaccagattcgccagcgtgtacgcctggaaccggaagagaatctctaactgcgtggccgattacagcgtgctctataactcggctagcttcagcacattcaagtgctacggcgtgagccccacaaagctgaacgacctgtgcttcaccaacgtctacgccgacagcttcgtgattagaggcgatgaggtccgacagatcgcccctggccaaaccggcaagattgctgactacaactacaagctgcctgatgacttcactggatgtgtgatcgcttggaactccaacaacctggactctaaagtgggcggaaactacaactaccggtaccggctgtttagaaagagtaaccttaaacctttcgagagagatatcagcacagaaatctaccaggctggcagcacaccttgtaacggcgtgcaaggcttcaactgctatttccctctccagtcttatggcttccagcctaccaacggcgtgggctatcagccctaccgagtggtggtgctgtccttcgagctgctgcatgcccctgctaccgtgtgcggccctaagaaatcgaccaacctggtgaagaacaagtgcgtgaattttaatttcaacggcctcaccggcaccggagtgctgaccgagagcaacaagaagttcctgcccttccagcagttcggaagagacatcgccgataccacagacgccgtgcgggacccccaaacactggaaatcctggacatcacaccttgcagcttcggcggcgtgagcgtgatcacccctggcaccaacacaagcaaccaggtggccgtgctctaccagggcgtgaactgcaccgaagtgccagtggccatccacgccgatcagctgacccctacctggagagtgtacagcaccggcagcaacgtgttccagacaagggctggttgtctgatcggcgccgagcacgtgaataattcctacgagtgcgacatccctattggcgccggaatctgtgccagctaccagacacagacaaactccccacgtagagccagatccgtcgccagccagagcatcatcgcttacaccatgagcctgggcgctgaaaacagcgtggcttacagcaacaattctatcgccatacctaccaattttacaatctcggtgacaaccgagatcctgcctgttagcatgaccaagaccagcgtggactgcacaatgtacatctgcggagacagcaccgagtgctccaacctgctgcttcaatacgggtccttctgtacacagctgaatagagccctgacaggcatcgctgttgagcaggacaagaacacccaggaggtgtttgcccaagtgaagcagatctacaagactccgcctatcaaggacttcggcggcttcaacttcagccagatcctgccagatccttctaagcctagcaagcgcagtttcatcgaggacctgttgttcaacaaggtgaccctggccgacgccggctttatcaagcagtacggcgattgcctgggcgacatcgccgctagagatctgatctgcgcccagaagttcaatggactgacagtgctgccgcccctgctgaccgatgagatgatcgctcagtacacctctgccctgctggccgggacaatcaccagcggatggacattcggggccggcgccgccctgcagatcccctttgccatgcagatggcctacagattcaacggtattggcgtgacccaaaacgtgctgtacgagaatcagaagttaatcgcaaaccagttcaacagcgccatcggcaagatccaggattccctgagttccacggccagcgctctgggtaagctgcaagacgtggtgaaccagaacgcacaggccctgaacaccctggtcaaacagctgagctccaacttcggagcgatcagcagcgtgcttaatgacatcctgagcagactggatccccccgaggccgaagtccaaatcgaccggctgatcacaggcaggttgcagagcctgcagacctacgtgacccaacagctgatcagagcagccgagatcagagcctcagccaatctggctgctacgaagatgagcgagtgtgtgctgggacagagcaagcgggtggatttttgcggcaaagggtaccacctgatgagcttccctcagagcgcccctcacggcgttgtgttcctgcacgtgacgtacgtgcccgcccaagagaagaacttcaccacagcccctgccatctgccacgacggaaaagcccacttccctcgtgagggcgtcttcgtgagcaacggcacacactggttcgtgactcagagaaacttctacgagcctcagatcatcaccaccgacaacacctttgtgagcggcaactgcgacgtggtgatcgggatcgtgaacaacaccgtgtacgaccccctgcagcctgagctggatagcttcaaagaggaactggacaagtatttcaagaatcacacctctccagacgtggacctgggcgacatcagcggcattaacgcctctgtggtgaacatccagaaggaaatcgatcggctgaacgaggtggccaagaacttgaacgagagcctgatcgacctgcaggagctgggcaagtacgagcagtacatcaagtggccttggtacatctggctgggattcatcgccggcctgattgccatcgtcatggtgaccatcatgctgtgttgcatgacaagctgctgcagctgtctgaagggatgttgctcttgtggctcttgctgtaaattcgacgaagacgactcggaacccgtgctgaagggcgttaagctccactacacctgatgagctcgctttcttgctgtccaatttctattaaaggttcctttgttccctaagtccaactactaaactgggggatattatgaagggccttgagcatctggattctgcctaataaaaaacatttattttcattgcaattgccatgtgtatgtgggttcgcccacatactctgatgatccccaatcgtggcgtgtcggcctgcttcggcaggcactggcgccgggatcattcatggcaactcgagctggtactgcatgcacgcaatgctagctgcccctttcccgtcctgggtaccccgagtctcccccgacctcgggtcccaggtatgctcccacctccacctgccccactcaccacctctgctagttccagacacctcc

SEQ ID NO: 6 - RNA, 4411 nt, synthetic construct
  source 1..4411: mol_type = other RNA
gggagacccaagctggctagcgtttaaacttaagcttggtaccgagctcggatccactagtccagtgtggtggaattcgaataaactagtattcttctggtccccacagactcagagagaacccgccaccatgttcgtgttcctggtgctgctgcccttagtgagcagccagtgcgtcaacctaactactagaacacagctgcctcctgcctacacaaacagcttcaccagaggcgtgtattaccccgataaggtgttccggtcttctgtgctgcacagcacccaggacctgtttctgcctttcttcagcaatgtgacctggttccacgccatccacgtgtctggcacaaacggcacaaaaaggttcgacaaccccgttctgcctttcaatgacggcgtgtacttcgctagcacagaaaagagcaacatcatcagaggatggatcttcggaaccaccctggattccaagacacagtccctgttgatcgttaataatgccaccaatgtggtgatcaaggtgtgtgagttccagttttgcaacgatccttttctgggcgtgtattaccacaagaataacaaaagctggatggaaagcgagtttagagtatactctagcgccaacaactgcaccttcgagtacgtcagccagccttttctgatggacctggaaggcaagcagggcaacttcaagaatctgagagagttcgtgttcaaaaacattgacggatatttcaaaatctacagcaagcacacacctatcaatctggtgcgggacctgccacaggggtttagcgcattggagcctctggtcgatctgcctatcggcatcaacatcacccggttccagaccctgctagccctgcatagaagctatctgacccctggcgacagctcaagcggctggaccgccggcgccgccgcctactacgtgggctacctgcagcctagaacctttctgctgaagtacaacgagaacggcaccataaccgacgctgtggactgcgccctggaccccctgtctgaaaccaagtgcaccctgaagagctttaccgtggaaaagggcatctaccaaacaagcaatttccgggtgcagcctaccgagtctatcgtgcggtttcccaacatcaccaacctgtgcccattcggagaagtgttcaacgccaccagattcgccagcgtgtacgcctggaaccggaagagaatctctaactgcgtggccgattacagcgtgctctataactcggctagcttcagcacattcaagtgctacggcgtgagccccacaaagctgaacgacctgtgcttcaccaacgtctacgccgacagcttcgtgattagaggcgatgaggtccgacagatcgcccctggccaaaccggcaagattgctgactacaactacaagctgcctgatgacttcactggatgtgtgatcgcttggaactccaacaacctggactctaaagtgggcggaaactacaactaccggtaccggctgtttagaaagagtaaccttaaacctttcgagagagatatcagcacagaaatctaccaggctggcagcacaccttgtaacggcgtgcaaggcttcaactgctatttccctctccagtcttatggcttccagcctaccaacggcgtgggctatcagccctaccgagtggtggtgctgtccttcgagctgctgcatgcccctgctaccgtgtgcggccctaagaaatcgaccaacctggtgaagaacaagtgcgtgaattttaatttcaacggcctcaccggcaccggagtgctgaccgagagcaacaagaagttcctgcccttccagcagttcggaagagacatcgccgataccacagacgccgtgcgggacccccaaacactggaaatcctggacatcacaccttgcagcttcggcggcgtgagcgtgatcacccctggcaccaacacaagcaaccaggtggccgtgctctaccagggcgtgaactgcaccgaagtgccagtggccatccacgccgatcagctgacccctacctggagagtgtacagcaccggcagcaacgtgttccagacaagggctggttgtctgatcggcgccgagcacgtgaataattcctacgagtgcgacatccctattggcgccggaatctgtgccagctaccagacacagacaaactccccacgtagagccagatccgtcgccagccagagcatcatcgcttacaccatgagcctgggcgctgaaaacagcgtggcttacagcaacaattctatcgccatacctaccaattttacaatctcggtgacaaccgagatcctgcctgttagcatgaccaagaccagcgtggactgcacaatgtacatctgcggagacagcaccgagtgctccaacctgctgcttcaatacgggtccttctgtacacagctgaatagagccctgacaggcatcgctgttgagcaggacaagaacacccaggaggtgtttgcccaagtgaagcagatctacaagactccgcctatcaaggacttcggcggcttcaacttcagccagatcctgccagatccttctaagcctagcaagcgcagtttcatcgaggacctgttgttcaacaaggtgaccctggccgacgccggctttatcaagcagtacggcgattgcctgggcgacatcgccgctagagatctgatctgcgcccagaagttcaatggactgacagtgctgccgcccctgctgaccgatgagatgatcgctcagtacacctctgccctgctggccgggacaatcaccagcggatggacattcggggccggcgccgccctgcagatcccctttgccatgcagatggcctacagattcaacggtattggcgtgacccaaaacgtgctgtacgagaatcagaagttaatcgcaaaccagttcaacagcgccatcggcaagatccaggattccctgagttccacggccagcgctctgggtaagctgcaagacgtggtgaaccagaacgcacaggccctgaacaccctggtcaaacagctgagctccaacttcggagcgatcagcagcgtgcttaatgacatcctgagcagactggatccccccgaggccgaagtccaaatcgaccggctgatcacaggcaggttgcagagcctgcagacctacgtgacccaacagctgatcagagcagccgagatcagagcctcagccaatctggctgctacgaagatgagcgagtgtgtgctgggacagagcaagcgggtggatttttgcggcaaagggtaccacctgatgagcttccctcagagcgcccctcacggcgttgtgttcctgcacgtgacgtacgtgcccgcccaagagaagaacttcaccacagcccctgccatctgccacgacggaaaagcccacttccctcgtgagggcgtcttcgtgagcaacggcacacactggttcgtgactcagagaaacttctacgagcctcagatcatcaccaccgacaacacctttgtgagcggcaactgcgacgtggtgatcgggatcgtgaacaacaccgtgtacgaccccctgcagcctgagctggatagcttcaaagaggaactggacaagtatttcaagaatcacacctctccagacgtggacctgggcgacatcagcggcattaacgcctctgtggtgaacatccagaaggaaatcgatcggctgaacgaggtggccaagaacttgaacgagagcctgatcgacctgcaggagctgggcaagtacgagcagtacatcaagtggccttggtacatctggctgggattcatcgccggcctgattgccatcgtcatggtgaccatcatgctgtgttgcatgacaagctgctgcagctgtctgaagggatgttgctcttgtggctcttgctgtaaattcgacgaagacgactcggaacccgtgctgaagggcgttaagctccactacacctgatgagctcgctttcttgctgtccaatttctattaaaggttcctttgttccctaagtccaactactaaactgggggatattatgaagggccttgagcatctggattctgcctaataaaaaacatttattttcattgcaattgccatgtgtatgtgggttcgcccacatactctgatgatccccaatcgtggcgtgtcggcctgcttcggcaggcactggcgccgggatcattcatggcaagctggagcctcggtggccatgcttcttgccccttgggcctccccccagcccctcctccccttcctgcacccgtacccccgtggtctttgaataaagtctgagtgggcggcaaaaaaaaaaaaaaaaaaaaaaaaaaaaaaagcatatgactaaaaaaaaaaaaaaaaaaaaaaaaaaaaaaaaaaaaaaaaaaaaaaaaaaaaaaaaaaaaaaaaaaaaaa

SEQ ID NO: 7 - protein, 1273 aa, synthetic construct
MFVFLVLLPLVSSQCVNLTTRTQLPPAYTNSFTRGVYYPDKVFRSSVLHSTQDLFLPFFSNVTWFHAIHVSGTNGTKRFDNPVLPFNDGVYFASTEKSNIIRGWIFGTTLDSKTQSLLIVNNATNVVIKVCEFQFCNDPFLGVYYHKNNKSWMESEFRVYSSANNCTFEYVSQPFLMDLEGKQGNFKNLREFVFKNIDGYFKIYSKHTPINLVRDLPQGFSALEPLVDLPIGINITRFQTLLALHRSYLTPGDSSSGWTAGAAAYYVGYLQPRTFLLKYNENGTITDAVDCALDPLSETKCTLKSFTVEKGIYQTSNFRVQPTESIVRFPNITNLCPFGEVFNATRFASVYAWNRKRISNCVADYSVLYNSASFSTFKCYGVSPTKLNDLCFTNVYADSFVIRGDEVRQIAPGQTGKIADYNYKLPDDFTGCVIAWNSNNLDSKVGGNYNYRYRLFRKSNLKPFERDISTEIYQAGSTPCNGVQGFNCYFPLQSYGFQPTNGVGYQPYRVVVLSFELLHAPATVCGPKKSTNLVKNKCVNFNFNGLTGTGVLTESNKKFLPFQQFGRDIADTTDAVRDPQTLEILDITPCSFGGVSVITPGTNTSNQVAVLYQGVNCTEVPVAIHADQLTPTWRVYSTGSNVFQTRAGCLIGAEHVNNSYECDIPIGAGICASYQTQTNSPRRARSVASQSIIAYTMSLGAENSVAYSNNSIAIPTNFTISVTTEILPVSMTKTSVDCTMYICGDSTECSNLLLQYGSFCTQLNRALTGIAVEQDKNTQEVFAQVKQIYKTPPIKDFGGFNFSQILPDPSKPSKRSFIEDLLFNKVTLADAGFIKQYGDCLGDIAARDLICAQKFNGLTVLPPLLTDEMIAQYTSALLAGTITSGWTFGAGAALQIPFAMQMAYRFNGIGVTQNVLYENQKLIANQFNSAIGKIQDSLSSTASALGKLQDVVNQNAQALNTLVKQLSSNFGAISSVLNDILSRLDPPEAEVQIDRLITGRLQSLQTYVTQQLIRAAEIRASANLAATKMSECVLGQSKRVDFCGKGYHLMSFPQSAPHGVVFLHVTYVPAQEKNFTTAPAICHDGKAHFPREGVFVSNGTHWFVTQRNFYEPQIITTDNTFVSGNCDVVIGIVNNTVYDPLQPELDSFKEELDKYFKNHTSPDVDLGDISGINASVVNIQKEIDRLNEVAKNLNESLIDLQELGKYEQYIKWPWYIWLGFIAGLIAIVMVTIMLCCMTSCCSCLKGCCSCGSCCKFDEDDSEPVLKGVKLHYT

SEQ ID NO: 8 - DNA, 4346 bp, COVID 19
  source 1..4346: mol_type = genomic DNA
gggagacccaagctggctagcgtttaaacttaagcttggtaccgagctcggatccactagtccagtgtggtggaattcagaataaactagtattcttctggtccccacagactcagagagaacccgccaccatgtttgtttttcttgttttattgccactagtctctagtcagtgtgttaatcttataaccagaactcaatcatacactaattctttcacacgtggtgtttattaccctgacaaagttttcagatcctcagttttacattcaactcaggacttgttcttacctttcttttccaatgttacttggttccatgctatctctgggaccaatggtactaagaggtttgataaccctgtcctaccatttaatgatggtgtttattttgcttccactgagaagtctaacataataagaggctggatttttggtactactttagattcgaagacccagtccctacttattgttaataacgctactaatgttgttattaaagtctgtgaatttcaattttgtaatgatccatttttggatgtttattaccacaaaaacaacaaaagttggatggaaagtgagttcagagtttattctagtgcgaataattgcacttttgaatatgtctctcagccttttcttatggaccttgaaggaaaacagggtaatttcaaaaatcttagggaatttgtgtttaagaatattgatggttattttaaaatatattctaagcacacgcctattaatttagggcgtgatctccctcagggtttttcggctttagaaccattggtagatttgccaataggtattaacatcactaggtttcaaactttacttgctttacatagaagttatttgactcctggtgattcttcttcaggttggacagctggtgctgcagcttattatgtgggttatcttcaacctaggacttttctattaaaatataatgaaaatggaaccattacagatgctgtagactgtgcacttgaccctctctcagaaacaaagtgtacgttgaaatccttcactgtagaaaaaggaatctatcaaacttctaactttagagtccaaccaacagaatctattgttagatttcctaatattacaaacttgtgcccttttgatgaagtttttaacgccaccagatttgcatctgtttatgcttggaacaggaagagaatcagcaactgtgttgctgattattctgtcctatataatttcgcaccatttttcgcttttaagtgttatggagtgtctcctactaaattaaatgatctctgctttactaatgtctatgcagattcatttgtaattagaggtaatgaagtcagccaaatcgctccagggcaaactggaaatattgctgattataattataaattaccagatgattttacaggctgcgttatagcttggaattctaacaagcttgattctaaggttggtggtaattataattaccggtatagattgtttaggaagtctaatctcaaaccttttgagagagatatttcaactgaaatctatcaggccggtaacaaaccttgtaatggtgttgcaggtgttaattgttactttcctttacaatcatatggtttccgacccacttatggtgttggtcaccaaccatacagagtagtagtactttcttttgaacttctacatgcaccagcaactgtttgtggacctaaaaagtctactaatttggttaaaaacaaatgtgtcaatttcaacttcaatggtttaacaggcacaggtgttcttactgagtctaacaaaaagtttctgcctttccaacaatttggcagagacattgctgacactactgatgctgtccgtgatccacagacacttgagattcttgacattacaccatgttcttttggtggtgtcagtgttataacaccaggaacaaatacttctaaccaggttgctgttctttatcagggtgttaactgcacagaagtccctgttgctattcatgcagatcaacttactcctacttggcgtgtttattctacaggttctaatgtttttcaaacacgtgcaggctgtttaataggggctgaatatgtcaacaactcatatgagtgtgacatacccattggtgcaggtatatgcgctagttatcagactcagactaagtctcatcggcgggcacgtagtgtagctagtcaatccatcattgcctacactatgtcacttggtgcagaaaattcagttgcttactctaataactctattgccatacccacaaattttactattagtgttaccacagaaattctaccagtgtctatgaccaagacatcagtagattgtacaatgtacatttgtggtgattcaactgaatgcagcaatcttttgttgcaatatggcagtttttgtacacaattaaaacgtgctttaactggaatagctgttgaacaagacaaaaacacccaagaagtttttgcacaagtcaaacaaatttacaaaacaccaccaattaaatattttggtggttttaatttttcacaaatattaccagatccatcaaaaccaagcaagaggtcatttattgaagatctacttttcaacaaagtgacacttgcagatgctggcttcatcaaacaatatggtgattgccttggtgatattgctgctagagacctcatttgtgcacaaaagtttaacggccttactgttttgccacctttgctcacagatgaaatgattgctcaatacacttctgcactgttagcgggtacaatcacttctggttggacctttggtgcaggtgctgcattacaaataccatttgctatgcaaatggcttataggtttaatggtattggagttacacagaatgttctctatgagaaccaaaaattgattgccaaccaatttaatagtgctattggcaaaattcaagactcactttcttccacagcaagtgcacttggaaaacttcaagatgtggtcaaccataatgcacaagctttaaacacgcttgttaaacaacttagctccaaatttggtgcaatttcaagtgttttaaatgatatcctttcacgtcttgacaaagttgaggctgaagtgcaaattgataggttgatcacaggcagacttcaaagtttgcagacatatgtgactcaacaattaattagagctgcagaaatcagagcttctgctaatcttgctgctactaaaatgtcagagtgtgtacttggacaatcaaaaagagttgatttttgtggaaagggctatcatcttatgtccttccctcagtcagcacctcatggtgtagtcttcttgcatgtgacttatgtccctgcacaagaaaagaacttcacaactgctcctgccatttgtcatgatggaaaagcacactttcctcgtgaaggtgtctttgtttcaaatggcacacactggtttgtaacacaaaggaatttttatgaaccacaaatcattactacagacaacacatttgtgtctggtaactgtgatgttgtaataggaattgtcaacaacacagtttatgatcctttgcaacctgaattagattcattcaaggaggagttagataaatattttaagaatcatacatcaccagatgttgatttaggtgacatctctggcattaatgcttcagttgtaaacattcaaaaagaaattgaccgcctcaatgaggttgccaagaatttaaatgaatctctcatcgatctccaagaacttggaaagtatgagcagtatataaaatggccatggtacatttggctaggttttatagctggcttgattgccatagtaatggtgacaattatgctttgctgtatgaccagttgctgtagttgtctcaagggctgttgttcttgtggatcctgctgcaaatttgatgaagacgactctgagccagtgctcaaaggagtcaaattacattacacatgatgactcgagctggtactgcatgcacgcaatgctagctgcccctttcccgtcctgggtaccccgagtctcccccgacctcgggtcccaggtatgctcccacctccacctgccccactcaccacctctgctagttccagacacctcccaagcacgcagcaatgcagctcaaaacgcttagcctagccacacccccacgggaaacagcagtgattaacctttagcaataaacgaaagtttaactaagctatactaaccccagggttggtcaatttcgtgccagccacaccctggagctagcaaaaaaaaaaaaaaaaaaaaaaaaaaaaaagcatatgactaaaaaaaaaaaaaaaaaaaaaaaaaaaaaaaaaaaaaaaaaaaaaaaaaaaaaaaaaaaaaaaaaaaaaa

SEQ ID NO: 9 - DNA, 4159 bp, synthetic construct
  source 1..4159: mol_type = other DNA
gggagacccaagctggctagcgtttaaacttaagcttggtaccgagctcggatccactagtccagtgtggtggaattcgggaaataagagagaaaagaagagtaagaagaaatataagagccaccatgttcgtttttttagttttattacctttagtgagcagccagtgcgtgaacctgatcacccggacccagagctacaccaacagcttcacccggggcgtgtactaccccgacaaggtgttccggagcagcgtgctgcacagcacccaggacctgttcctgcccttcttcagcaacgtgacctggttccacgccatcagcggcaccaacggcaccaagcggttcgacaaccccgtgctgcccttcaacgacggcgtgtacttcgccagcaccgagaagagcaacatcatccggggctggatcttcggcaccaccctggacagcaagacccagagcctgctgatcgtgaacaacgccaccaacgtggtgatcaaggtgtgcgagttccagttctgcaacgaccccttcctggacgtgtactaccacaagaacaacaagagctggatggagagcgagttccgggtgtacagcagcgccaacaactgcaccttcgagtacgtgagccagcccttcctgatggacctggagggcaagcagggcaacttcaagaacctgcgggagttcgtgttcaagaacatcgacggctacttcaagatctacagcaagcacacccccatcaacctgggccgggacctgccccagggcttcagcgccctggagcccctggtggacctgcccatcggcatcaacatcacccggttccagaccctgctggccctgcaccggagctacctgacccccggcgacagcagcagcggctggaccgccggcgccgccgcctactacgtgggctacctgcagccccggaccttcctgctgaagtacaacgagaacggcaccatcaccgacgccgtggactgcgccctggaccccctgagcgagaccaagtgcaccctgaagagcttcaccgtggagaagggcatctaccagaccagcaacttccgggtgcagcccaccgagagcatcgtgcggttccccaacatcaccaacctgtgccccttcgacgaggtgttcaacgccacccggttcgccagcgtgtacgcctggaaccggaagcggatcagcaactgcgtggccgactacagcgtgctgtacaacttcgcccccttcttcgccttcaagtgctacggcgtgagccccaccaagctgaacgacctgtgcttcaccaacgtgtacgccgacagcttcgtgatccggggcaacgaggtgagccagatcgcccccggccagaccggcaacatcgccgactacaactacaagctgcccgacgacttcaccggctgcgtgatcgcctggaacagcaacaagctggacagcaaggtgggcggcaactacaactaccggtaccggctgttccggaagagcaacctgaagcccttcgagcgggacatcagcaccgagatctaccaggccggcaacaagccctgcaacggcgtggccggcgtgaactgctacttccccctgcagagctacggcttccggcccacctacggcgtgggccaccagccctaccgggtggtggtgctgagcttcgagctgctgcacgcccccgccaccgtgtgcggccccaagaagagcaccaacctggtgaagaacaagtgcgtgaacttcaacttcaacggcctgaccggcaccggcgtgctgaccgagagcaacaagaagttcctgcccttccagcagttcggccgggacatcgccgacaccaccgacgccgtgcgggacccccagaccctggagatcctggacatcaccccctgcagcttcggcggcgtgagcgtgatcacccccggcaccaacaccagcaaccaggtggccgtgctgtaccagggcgtgaactgcaccgaggtgcccgtggccatccacgccgaccagctgacccccacctggcgggtgtacagcaccggcagcaacgtgttccagacccgcgccggctgcctgatcggcgccgagtacgtgaacaacagctacgagtgcgacatccccatcggcgccggcatctgcgcctcctaccagacccagaccaagagccaccggcgggcccggagcgtggccagccagagcatcatcgcctacaccatgagcctgggcgccgagaacagcgtggcctacagcaacaacagcatcgccatccccaccaacttcaccatcagcgtgaccaccgagatcctgcccgtgagcatgaccaagaccagcgtggactgcaccatgtacatctgcggcgacagcaccgagtgcagcaacctgctgctgcagtacggcagcttctgcacccagctgaagcgggccctgaccggcatcgccgtggagcaggacaagaacacccaggaggtgttcgcccaggtgaagcagatctacaagaccccccccatcaagtacttcggcggcttcaacttcagccagatcctgcccgaccccagcaagcccagcaagcggagcttcatcgaggacctgctgttcaacaaggtgaccctggccgacgccggcttcatcaagcagtacggcgactgcctgggcgacatcgccgcccgggacctgatctgcgcccagaagttcaacggcctgaccgtgctgccccccctgctgaccgacgagatgatcgcccagtacaccagcgccctgctggccggcaccatcaccagcggctggaccttcggcgccggcgccgccctgcagatccccttcgccatgcagatggcctaccggttcaacggcatcggcgtgacccagaacgtgctgtacgagaaccagaagctgatcgccaaccagttcaacagcgccatcggcaagatccaggacagcctgagcagcaccgccagcgccctgggcaagctgcaggacgtggtgaaccacaacgcccaggccctgaacaccctggtgaagcagctgagcagcaagttcggcgccatcagcagcgtgctgaacgacatcctgagccggctggacccccccgaggccgaggtgcagatcgaccggctgatcaccggccggctgcagagcctgcagacctacgtgacccagcagctgatccgggccgccgagatccgggccagcgccaacctggccgccaccaagatgagcgagtgcgtgctgggccagagcaagcgggtggacttctgcggcaagggctaccacctgatgagcttcccccagagcgccccccacggcgtggtgttcctgcacgtgacctacgtgcccgcccaggagaagaacttcaccaccgcccccgccatctgccacgacggcaaggcccacttcccccgggagggcgtgttcgtgagcaacggcacccactggttcgtgacccagcggaacttctacgagccccagatcatcaccaccgacaacaccttcgtgagcggcaactgcgacgtggtgatcggcatcgtgaacaacaccgtgtacgaccccctgcagcccgagctggacagcttcaaggaggagctggacaagtacttcaagaaccacaccagccccgacgtggacctgggcgacatcagcggcatcaacgccagcgtggtgaacatccagaaggagatcgaccggctgaacgaggtggccaagaacctgaacgagagcctgatcgacctgcaggagctgggcaagtacgagcagtacatcaagtggccctggtacatctggctgggcttcatcgccggcctgatcgccatcgtgatggtgaccatcatgctgtgctgcatgaccagctgctgcagctgcctgaagggctgctgcagctgcggcagctgctgcaagttcgacgaggacgacagcgagcccgtgctgaagggcgtgaagctgcactacacctgataataggctggagcctcggtggccatgcttcttgccccttgggcctccccccagcccctcctccccttcctgcacccgtacccccgtggtctttgaataaagtctgagtgggcggcaaaaaaaaaaaaaaaaaaaaaaaaaaaaaaagcatatgactaaaaaaaaaaaaaaaaaaaaaaaaaaaaaaaaaaaaaaaaaaaaaaaaaaaaaaaaaaaaaaaaaaaaaa

SEQ ID NO: 10 - DNA, 4159 bp, synthetic construct
  source 1..4159: mol_type = other DNA
gggagacccaagctggctagcgtttaaacttaagcttggtaccgagctcggatccactagtccagtgtggtggaattcgggaaataagagagaaaagaagagtaagaagaaatataagagccaccatgttcgtttttttagttttattacctttagtgagcagccagtgcgtgaacctgatcacccggacccagagctacaccaacagcttcacccggggcgtgtactaccccgacaaggtgttccggagcagcgtgctgcacagcacccaggacctgttcctgcccttcttcagcaacgtgacctggttccacgccatcagcggcaccaacggcaccaagcggttcgacaaccccgtgctgcccttcaacgacggcgtgtacttcgccagcaccgagaagagcaacatcatccggggctggatcttcggcaccaccctggacagcaagacccagagcctgctgatcgtgaacaacgccaccaacgtggtgatcaaggtgtgcgagttccagttctgcaacgaccccttcctggacgtgtactaccacaagaacaacaagagctggatggagagcgagttccgggtgtacagcagcgccaacaactgcaccttcgagtacgtgagccagcccttcctgatggacctggagggcaagcagggcaacttcaagaacctgcgggagttcgtgttcaagaacatcgacggctacttcaagatctacagcaagcacacccccatcaacctgggccgggacctgccccagggcttcagcgccctggagcccctggtggacctgcccatcggcatcaacatcacccggttccagaccctgctggccctgcaccggagctacctgacccccggcgacagcagcagcggctggaccgccggcgccgccgcctactacgtgggctacctgcagccccggaccttcctgctgaagtacaacgagaacggcaccatcaccgacgccgtggactgcgccctggaccccctgagcgagaccaagtgcaccctgaagagcttcaccgtggagaagggcatctaccagaccagcaacttccgggtgcagcccaccgagagcatcgtgcggttccccaacatcaccaacctgtgccccttcgacgaggtgttcaacgccacccggttcgccagcgtgtacgcctggaaccggaagcggatcagcaactgcgtggccgactacagcgtgctgtacaacttcgcccccttcttcgccttcaagtgctacggcgtgagccccaccaagctgaacgacctgtgcttcaccaacgtgtacgccgacagcttcgtgatccggggcaacgaggtgagccagatcgcccccggccagaccggcaacatcgccgactacaactacaagctgcccgacgacttcaccggctgcgtgatcgcctggaacagcaacaagctggacagcaaggtgggcggcaactacaactaccggtaccggctgttccggaagagcaacctgaagcccttcgagcgggacatcagcaccgagatctaccaggccggcaacaagccctgcaacggcgtggccggcgtgaactgctacttccccctgcagagctacggcttccggcccacctacggcgtgggccaccagccctaccgggtggtggtgctgagcttcgagctgctgcacgcccccgccaccgtgtgcggccccaagaagagcaccaacctggtgaagaacaagtgcgtgaacttcaacttcaacggcctgaccggcaccggcgtgctgaccgagagcaacaagaagttcctgcccttccagcagttcggccgggacatcgccgacaccaccgacgccgtgcgggacccccagaccctggagatcctggacatcaccccctgcagcttcggcggcgtgagcgtgatcacccccggcaccaacaccagcaaccaggtggccgtgctgtaccagggcgtgaactgcaccgaggtgcccgtggccatccacgccgaccagctgacccccacctggcgggtgtacagcaccggcagcaacgtgttccagacccgggccggctgcctgatcggcgccgagtacgtgaacaacagctacgagtgcgacatccccatcggcgccggcatctgcgccagctaccagacccagaccaagagccaccggcgggcccggagcgtggccagccagagcatcatcgcctacaccatgagcctgggcgccgagaacagcgtggcctacagcaacaacagcatcgccatccccaccaacttcaccatcagcgtgaccaccgagatcctgcccgtgagcatgaccaagaccagcgtggactgcaccatgtacatctgcggcgacagcaccgagtgctccaacctgctgctgcagtacggcagcttctgcacccagctgaagcgggccctgaccggcatcgccgtggagcaggacaagaacacccaggaggtgttcgcccaggtgaagcagatctacaagaccccccccatcaagtacttcggcggcttcaacttcagccagatcctgcccgaccccagcaagcccagcaagcgcagcttcatcgaggacctgctgttcaacaaggtgaccctggccgacgccggcttcatcaagcagtacggcgactgcctgggcgacatcgccgcccgggacctgatctgcgcccagaagttcaacggcctgaccgtgctgccccccctgctgaccgacgagatgatcgcccagtacaccagcgccctgctggccggcaccatcaccagcggctggaccttcggcgccggcgccgccctgcagatccccttcgccatgcagatggcctaccggttcaacggcatcggcgtgacccagaacgtgctgtacgagaaccagaagctgatcgccaaccagttcaacagcgccatcggcaagatccaggacagcctgagcagcaccgccagcgccctgggcaagctgcaggacgtggtgaaccacaacgcccaggccctgaacaccctggtgaagcagctgagcagcaagttcggcgccatcagcagcgtgctgaacgacatcctgagccggctggacccccccgaggccgaggtgcagatcgaccggctgatcaccggccggctgcagagcctgcagacctacgtgacccagcagctgatccgggccgccgagatccgggccagcgccaacctggccgccaccaagatgagcgagtgcgtgctgggccagagcaagcgggtggacttctgcggcaagggctaccacctgatgagcttcccccagagcgccccccacggcgtggtgttcctgcacgtgacctacgtgcccgcccaggagaagaacttcaccaccgcccccgccatctgccacgacggcaaggcccacttcccccgggagggcgtgttcgtgagcaacggcacccactggttcgtgacccagcggaacttctacgagccccagatcatcaccaccgacaacaccttcgtgagcggcaactgcgacgtggtgatcggcatcgtgaacaacaccgtgtacgaccccctgcagcccgagctggacagcttcaaggaggagctggacaagtacttcaagaaccacaccagccccgacgtggacctgggcgacatcagcggcatcaacgccagcgtggtgaacatccagaaggagatcgaccggctgaacgaggtggccaagaacctgaacgagagcctgatcgacctgcaggagctgggcaagtacgagcagtacatcaagtggccctggtacatctggctgggcttcatcgccggcctgatcgccatcgtgatggtgaccatcatgctgtgctgcatgaccagctgctgcagctgcctgaagggctgctgcagctgcggcagctgctgcaagttcgacgaggacgacagcgagcccgtgctgaagggcgtgaagctgcactacacctgataataggctggagcctcggtggccatgcttcttgccccttgggcctccccccagcccctcctccccttcctgcacccgtacccccgtggtctttgaataaagtctgagtgggcggcaaaaaaaaaaaaaaaaaaaaaaaaaaaaaaagcatatgactaaaaaaaaaaaaaaaaaaaaaaaaaaaaaaaaaaaaaaaaaaaaaaaaaaaaaaaaaaaaaaaaaaaaaa

SEQ ID NO: 11 - DNA, 4346 bp, synthetic construct
  source 1..4346: mol_type = other DNA
gggagacccaagctggctagcgtttaaacttaagcttggtaccgagctcggatccactagtccagtgtggtggaattcagaataaactagtattcttctggtccccacagactcagagagaacccgccaccatgttcgtttttttagttttattacctttagtgagcagccagtgcgtgaacctgatcacccggacccagagctacaccaacagcttcacccggggcgtgtactaccccgacaaggtgttccggagcagcgtgctgcacagcacccaggacctgttcctgcccttcttcagcaacgtgacctggttccacgccatcagcggcaccaacggcaccaagcggttcgacaaccccgtgctgcccttcaacgacggcgtgtacttcgccagcaccgagaagagcaacatcatccggggctggatcttcggcaccaccctggacagcaagacccagagcctgctgatcgtgaacaacgccaccaacgtggtgatcaaggtgtgcgagttccagttctgcaacgaccccttcctggacgtgtactaccacaagaacaacaagtcctggatggagagcgagttccgggtgtacagcagcgccaacaactgcaccttcgagtacgtgagccagcccttcctgatggacctggagggcaagcagggcaacttcaagaacctgcgggagttcgtgttcaagaacatcgacggctacttcaagatctacagcaagcacacccccatcaacctgggccgggacctgccccagggcttcagcgccctggagcccctggtggacctgcccatcggcatcaacatcacccggttccagaccctgctggccctgcaccggagctacctgacccccggcgacagcagcagcggctggaccgccggcgccgccgcctactacgtgggctacctgcagccccggaccttcctgctgaagtacaacgagaacggcaccatcaccgacgccgtggactgcgccctggaccccctgagcgagaccaagtgcaccctgaagagcttcaccgtggagaagggcatctaccagaccagcaacttccgggtgcagcccaccgagagcatcgtgcggttccccaacatcaccaacctgtgccccttcgacgaggtgttcaacgccacccggttcgccagcgtgtacgcctggaaccggaagcggatcagcaactgcgtggccgactacagcgtgctgtacaacttcgcccccttcttcgccttcaagtgctacggcgtgagccccaccaagctgaacgacctgtgcttcaccaacgtgtacgccgacagcttcgtgatccggggcaacgaggtgagccagatcgcccccggccagaccggcaacatcgccgactacaactacaagctgcccgacgacttcaccggctgcgtgatcgcctggaacagcaacaagctggacagcaaggtgggcggcaactacaactaccggtaccggctgttccggaagagcaacctgaagcccttcgagcgggacatcagcaccgagatctaccaggccggcaacaagccctgcaacggcgtggccggcgtgaactgctacttccccctgcagagctacggcttccggcccacctacggcgtgggccaccagccctaccgggtggtggtgctgagcttcgagctgctgcacgcccccgccaccgtgtgcggccccaagaagagcaccaacctggtgaagaacaagtgcgtgaacttcaacttcaacggcctgaccggcaccggcgtgctgaccgagagcaacaagaagttcctgcccttccagcagttcggccgggacatcgccgacaccaccgacgccgtgcgggacccccagaccctggagatcctggacatcaccccctgcagcttcggcggcgtgtccgtgatcacccccggcaccaacaccagcaaccaggtggccgtgctgtaccagggcgtgaactgcaccgaggtgcccgtggccatccacgccgaccagctgacccccacctggcgggtgtacagcaccggcagcaacgtgttccagacccgggccggctgcctgatcggcgccgagtacgtgaacaacagctacgagtgcgacatccccatcggcgccggcatctgcgccagctaccagacccagaccaagagccaccggcgggcccggagcgtggccagccagagcatcatcgcctacaccatgagcctgggcgccgagaacagcgtggcctacagcaacaacagcatcgccatccccaccaacttcaccatcagcgtgaccaccgagatcctgcccgtgagcatgaccaagaccagcgtggactgcaccatgtacatctgcggcgacagcaccgagtgcagcaacctgctgctgcagtacggcagcttctgcacccagctgaagcgggccctgaccggcatcgccgtggagcaggacaagaacacccaggaggtgttcgcccaggtgaagcagatctacaagaccccccccatcaagtacttcggcggcttcaacttcagccagatcctgcccgaccccagcaagcccagcaagcggagcttcatcgaggacctgctgttcaacaaggtgaccctggccgacgccggcttcatcaagcagtacggcgactgcctgggcgacatcgccgcccgggacctgatctgcgcccagaagttcaacggcctgaccgtgctgccccccctgctgaccgacgagatgatcgcccagtacaccagcgccctgctggccggcaccatcaccagcggctggaccttcggcgccggcgccgccctgcagatccccttcgccatgcagatggcctaccggttcaacggcatcggcgtgacccagaacgtgctgtacgagaaccagaagctgatcgccaaccagttcaacagcgccatcggcaagatccaggacagcctgagcagcaccgccagcgccctgggcaagctgcaggacgtggtgaaccacaacgcccaggccctgaacaccctggtgaagcagctgagcagcaagttcggcgccatcagcagcgtgctgaacgacatcctgagccggctggacccccccgaggccgaggtgcagatcgaccggctgatcaccggccggctgcagagcctgcagacctacgtgacccagcagctgatccgggccgccgagatccgggccagcgccaacctggccgccaccaagatgagcgagtgcgtgctgggccagagcaagcgggtggacttctgcggcaagggctaccacctgatgagcttcccccagagcgccccccacggcgtggtgttcctgcacgtgacctacgtgcccgcccaggagaagaacttcaccaccgcccccgccatctgccacgacggcaaggcccacttcccccgggagggcgtgttcgtgagcaacggcacccactggttcgtgacccagcggaacttctacgagccccagatcatcaccaccgacaacaccttcgtgagcggcaactgcgacgtggtgatcggcatcgtgaacaacaccgtgtacgaccccctgcagcccgagctggacagcttcaaggaggagctggacaagtacttcaagaaccacaccagccccgacgtggacctgggcgacatcagcggcatcaacgccagcgtggtgaacatccagaaggagatcgaccggctgaacgaggtggccaagaacctgaacgagagcctgatcgacctgcaggagctgggcaagtacgagcagtacatcaagtggccctggtacatctggctgggcttcatcgccggcctgatcgccatcgtgatggtgaccatcatgctgtgctgcatgaccagctgctgcagctgcctgaagggctgctgcagctgcggcagctgctgcaagttcgacgaggacgacagcgagcccgtgctgaagggcgtgaagctgcactacacctgatgactcgagctggtactgcatgcacgcaatgctagctgcccctttcccgtcctgggtaccccgagtctcccccgacctcgggtcccaggtatgctcccacctccacctgccccactcaccacctctgctagttccagacacctcccaagcacgcagcaatgcagctcaaaacgcttagcctagccacacccccacgggaaacagcagtgattaacctttagcaataaacgaaagtttaactaagctatactaaccccagggttggtcaatttcgtgccagccacaccctggagctagcaaaaaaaaaaaaaaaaaaaaaaaaaaaaaagcatatgactaaaaaaaaaaaaaaaaaaaaaaaaaaaaaaaaaaaaaaaaaaaaaaaaaaaaaaaaaaaaaaaaaaaaaa

SEQ ID NO: 12 - DNA, 4346 bp, synthetic construct
  source 1..4346: mol_type = other DNA
gggagacccaagctggctagcgtttaaacttaagcttggtaccgagctcggatccactagtccagtgtggtggaattcagaataaactagtattcttctggtccccacagactcagagagaacccgccaccatgttcgtttttttagttttattaccattagtgagcagccagtgcgtgaacctgatcacccggacccagagctacaccaacagcttcacccggggcgtgtactaccccgacaaggtgttccggagcagcgtgctgcacagcacccaggacctgttcctgcccttcttcagcaacgtgacctggttccacgccatcagcggcaccaacggcaccaagcggttcgacaaccccgtgctgcccttcaacgacggcgtgtacttcgccagcaccgagaagagcaacatcatccggggctggatcttcggcaccaccctggacagcaagacccagagcctgctgatcgtgaacaacgccaccaacgtggtgatcaaggtgtgcgagttccagttctgcaacgaccccttcctggacgtgtactaccacaagaacaacaagagctggatggagagcgagttccgggtgtacagcagcgccaacaactgcaccttcgagtacgtgagccagcccttcctgatggacctggagggcaagcagggcaacttcaagaacctgcgggagttcgtgttcaagaacatcgacggctacttcaagatctacagcaagcacacccccatcaacctgggccgggacctgccccagggcttcagcgccctggagcccctggtggacctgcccatcggcatcaacatcacccggttccagaccctgctggccctgcaccggagctacctgacccccggcgacagcagcagcggctggaccgccggcgccgccgcctactacgtgggctacctgcagccccggaccttcctgctgaagtacaacgagaacggcaccatcaccgacgccgtggactgcgccctggaccccctgagcgagaccaagtgcaccctgaagagcttcaccgtggagaagggcatctaccagaccagcaacttccgggtgcagcccaccgagagcatcgtgcggttccccaacatcaccaacctgtgccccttcgacgaggtgttcaacgccacccggttcgccagcgtgtacgcctggaaccggaagcggatcagcaactgcgtggccgactacagcgtgctgtacaacttcgcccccttcttcgccttcaagtgctacggcgtgagccccaccaagctgaacgacctgtgcttcaccaacgtgtacgccgacagcttcgtgatccggggcaacgaggtgagccagatcgcccccggccagaccggcaacatcgccgactacaactacaagctgcccgacgacttcaccggctgcgtgatcgcctggaacagcaacaagctggacagcaaggtgggcggcaactacaactaccggtaccggctgttccggaagagcaacctgaagcccttcgagcgggacatcagcaccgagatctaccaggccggcaacaagccctgcaacggcgtggccggcgtgaactgctacttccccctgcagagctacggcttccggcccacctacggcgtgggccaccagccctaccgggtggtggtgctgagcttcgagctgctgcacgcccccgccaccgtgtgcggccccaagaagagcaccaacctggtgaagaacaagtgcgtgaacttcaacttcaacggcctgaccggcaccggcgtgctgaccgagagcaacaagaagttcctgcccttccagcagttcggccgggacatcgccgacaccaccgacgccgtgcgggacccccagaccctggagatcctggacatcaccccctgcagcttcggcggcgtgagcgtgatcacccccggcaccaacaccagcaaccaggtggccgtgctgtaccagggcgtgaactgcaccgaggtgcccgtggccatccacgccgaccagctgacccccacctggcgggtgtacagcaccggcagcaacgtgttccagacccgggccggctgcctgatcggcgccgagtacgtgaacaacagctacgagtgcgacatccccatcggcgccggcatctgcgccagctaccagacccagaccaagagccaccggcgggcccggagcgtggccagccagagcatcatcgcctacaccatgagcctgggcgccgagaacagcgtggcctacagcaacaacagcatcgccatccccaccaacttcaccatcagcgtgaccaccgagatcctgcccgtgagcatgaccaagaccagcgtggactgcaccatgtacatctgcggcgacagcaccgagtgcagcaacctgctgctgcagtacggcagcttctgcacccagctgaagcgggccctgaccggcatcgccgtggagcaggacaagaacacccaggaggtgttcgcccaggtgaagcagatctacaagaccccccccatcaagtacttcggcggcttcaacttcagccagatcctgcccgaccccagcaagcccagcaagcggagcttcatcgaggacctgctgttcaacaaggtgaccctggccgacgccggcttcatcaagcagtacggcgactgcctgggcgacatcgccgcccgggacctgatctgcgcccagaagttcaacggcctgaccgtgctgccccccctgctgaccgacgagatgatcgcccagtacaccagcgccctgctggccggcaccatcaccagcggctggaccttcggcgccggcgccgccctgcagatccccttcgccatgcagatggcctaccggttcaacggcatcggcgtgacccagaacgtgctgtacgagaaccagaagctgatcgccaaccagttcaacagcgccatcggcaagatccaggacagcctgagcagcaccgccagcgccctgggcaagctgcaggacgtggtgaaccacaacgcccaggccctgaacaccctggtgaagcagctgagcagcaagttcggcgccatcagcagcgtgctgaacgacatcctgagccggctggacccccccgaggccgaggtgcagatcgaccggctgatcaccggccggctgcagagcctgcagacctacgtgacccagcagctgatccgggccgccgagatccgggccagcgccaacctggccgccaccaagatgagcgagtgcgtgctgggccagagcaagcgggtggacttctgcggcaagggctaccacctgatgtccttcccccagagcgccccccacggcgtggtgttcctgcacgtgacctacgtgcccgcccaggagaagaacttcaccaccgcccccgccatctgccacgacggcaaggcccacttcccccgggagggcgtgttcgtgagcaacggcacccactggttcgtgacccagcggaacttctacgagccccagatcatcaccaccgacaacaccttcgtgagcggcaactgcgacgtggtgatcggcatcgtgaacaacaccgtgtacgaccccctgcagcccgagctggacagcttcaaggaggagctggacaagtacttcaagaaccacaccagccccgacgtggacctgggcgacatcagcggcatcaacgccagcgtggtgaacatccagaaggagatcgaccggctgaacgaggtggccaagaacctgaacgagagcctgatcgacctgcaggagctgggcaagtacgagcagtacatcaagtggccctggtacatctggctgggcttcatcgccggcctgatcgccatcgtgatggtgaccatcatgctgtgctgcatgaccagctgctgcagctgcctgaagggctgctgcagctgcggcagctgctgcaagttcgacgaggacgacagcgagcccgtgctgaagggcgtgaagctgcactacacctgatgactcgagctggtactgcatgcacgcaatgctagctgcccctttcccgtcctgggtaccccgagtctcccccgacctcgggtcccaggtatgctcccacctccacctgccccactcaccacctctgctagttccagacacctcccaagcacgcagcaatgcagctcaaaacgcttagcctagccacacccccacgggaaacagcagtgattaacctttagcaataaacgaaagtttaactaagctatactaaccccagggttggtcaatttcgtgccagccacaccctggagctagcaaaaaaaaaaaaaaaaaaaaaaaaaaaaaagcatatgactaaaaaaaaaaaaaaaaaaaaaaaaaaaaaaaaaaaaaaaaaaaaaaaaaaaaaaaaaaaaaaaaaaaaaa

SEQ ID NO: 13 - DNA, 4295 bp, synthetic construct
  source 1..4295: mol_type = other DNA
gggagacccaagctggctagcgtttaaacttaagcttggtaccgagctcggatccactagtccagtgtggtggaattcagaataaactagtattcttctggtccccacagactcagagagaacccgccaccatgttcgtttttttagttttattacctttagtgagctcccagtgcgtgaacctgatcacccggacccagagctacaccaacagcttcacccggggcgtgtactaccccgacaaggtgttccggagcagcgtgctgcacagcacccaggacctgttcctgcccttcttcagcaacgtgacctggttccacgccatccacgtgagcggcaccaacggcaccaagcggttcgacaaccccgccctgcccttcaacgacggcgtgtacttcgccagcaccgagaagagcaacatcatccggggctggatcttcggcaccaccctggacagcaagacccagagcctgctgatcgtgaacaacgccaccaacgtggtgatcaaggtgtgcgagttccagttctgcaacgaccccttcctggacgtgtaccagaagaacaacaagagctggatggagagcgagttccgggtgtacagcagcgccaacaactgcaccttcgagtacgtgagccagcccttcctgatggacctggagggcaaggagggcaacttcaagaacctgcgggagttcgtgttcaagaacatcgacggctacttcaagatctacagcaagcacacccccatcaacctggagcgggacctgccccagggcttcagcgccctggagcccctggtggacctgcccatcggcatcaacatcacccggttccagaccctgctggccctgcaccggagctacctgacccccgtggacagcagcagcggctggaccgccggcgccgccgcctactacgtgggctacctgcagccccggaccttcctgctgaagtacaacgagaacggcaccatcaccgacgccgtggactgcgccctggaccccctgtccgagaccaagtgcaccctgaagagcttcaccgtggagaagggcatctaccagaccagcaacttccgggtgcagcccaccgagagcatcgtgcggttccccaacatcaccaacctgtgccccttccacgaggtgttcaacgccaccaccttcgccagcgtgtacgcctggaaccggaagcggatcagcaactgcgtggccgactacagcgtgatctacaacttcgcccccttcttcgccttcaagtgctacggcgtgagccccaccaagctgaacgacctgtgcttcaccaacgtgtacgccgacagcttcgtgatccggggcaacgaggtgagccagatcgcccccggccagaccggcaacatcgccgactacaactacaagctgcccgacgacttcaccggctgcgtgatcgcctggaacagcaacaagctggacagcaagcccagcggcaactacaactacctgtaccggctgttccggaagagcaagctgaagcccttcgagcgggacatcagcaccgagatctaccaggccggcaacaagccctgcaacggcgtggccggcagcaactgctacagccccctgcggagctacggcttccggcccacctacggcgtgggccaccagccctaccgggtggtggtgctgagcttcgagctgctgcacgcccccgccaccgtgtgcggccccaagaagagcaccaacctggtgaagaacaagtgcgtgaacttcaacttcaacggcctgaccggcaccggcgtgctgaccgagagcaacaagaagttcctgcccttccagcagttcggccgggacatcgccgacaccaccgacgccgtgcgggacccccagaccctggagatcctggacatcaccccctgcagcttcggcggcgtgagcgtgatcacccccggcaccaacaccagcaaccaggtggccgtgctgtaccagggcgtgaactgcaccgaggtgcccgtggccatccacgccgaccagctgacccccacctggcgggtgtacagcaccggcagcaacgtgttccagacccgggccggctgcctgatcggcgccgagtacgtgaacaacagctacgagtgcgacatccccatcggcgccggcatctgcgccagctaccagacccagaccaagagccaccggcgggcccggagcgtggccagccagagcatcatcgcctacaccatgagcctgggcgccgagaacagcgtggcctacagcaacaacagcatcgccatccccaccaacttcaccatcagcgtgaccaccgagatcctgcccgtgagcatgaccaagaccagcgtggactgcaccatgtacatctgcggcgacagcaccgagtgcagcaacctgctgctgcagtacggcagcttctgcacccagctgaagcgggccctgaccggcatcgccgtggagcaggacaagaacacccaggaggtgttcgcccaggtgaagcagatctacaagaccccccccatcaagtacttcggcggcttcaacttcagccagatcctgcccgaccccagcaagcccagcaagcggagcttcatcgaggacctgctgttcaacaaggtgaccctggccgacgccggcttcatcaagcagtacggcgactgcctgggcgacatcgccgcccgggacctgatctgcgcccagaagttcaacggcctgaccgtgctgccccccctgctgaccgacgagatgatcgcccagtacaccagcgccctgctggccggcaccatcaccagcggctggaccttcggcgccggcgccgccctgcagatccccttcgccatgcagatggcctaccggttcaacggcatcggcgtgacccagaacgtgctgtacgagaaccagaagctgatcgccaaccagttcaacagcgccatcggcaagatccaggacagcctgagcagcaccgccagcgccctgggcaagctgcaggacgtggtgaaccacaacgcccaggccctgaacaccctggtgaagcagctgagcagcaagttcggcgccatcagcagcgtgctgaacgacatcctgagccggctggacccccccgaggccgaggtgcagatcgaccggctgatcaccggccggctgcagagcctgcagacctacgtgacccagcagctgatccgggccgccgagatccgggccagcgccaacctggccgccaccaagatgagcgagtgcgtgctgggccagagcaagcgggtggacttctgcggcaagggctaccacctgatgagcttcccccagagcgccccccacggcgtggtgttcctgcacgtgacctacgtgcccgcccaggagaagaacttcaccaccgcccccgccatctgccacgacggcaaggcccacttcccccgggagggcgtgttcgtgagcaacggcacccactggttcgtgacccagcggaacttctacgagccccagatcatcaccaccgacaacaccttcgtgagcggcaactgcgacgtggtgatcggcatcgtgaacaacaccgtgtacgaccccctgcagcccgagctggacagcttcaaggaggagctggacaagtacttcaagaaccacaccagccccgacgtggacctgggcgacatcagcggcatcaacgccagcgtggtgaacatccagaaggagatcgaccggctgaacgaggtggccaagaacctgaacgagagcctgatcgacctgcaggagctgggcaagtacgagcagtacatcaagtggccctggtacatctggctgggcttcatcgccggcctgatcgccatcgtgatggtgaccatcatgctgtgctgcatgaccagctgctgcagctgcctgaagggctgctgcagctgcggcagctgctgcaagtgatgactcgagctggtactgcatgcacgcaatgctagctgcccctttcccgtcctgggtaccccgagtctcccccgacctcgggtcccaggtatgctcccacctccacctgccccactcaccacctctgctagttccagacacctcccaagcacgcagcaatgcagctcaaaacgcttagcctagccacacccccacgggaaacagcagtgattaacctttagcaataaacgaaagtttaactaagctatactaaccccagggttggtcaatttcgtgccagccacaccctggagctagcaaaaaaaaaaaaaaaaaaaaaaaaaaaaaagcatatgactaaaaaaaaaaaaaaaaaaaaaaaaaaaaaaaaaaaaaaaaaaaaaaaaaaaaaaaaaaaaaaaaaaaaaa

SEQ ID NO: 14 - DNA, 4295 bp, synthetic construct
  source 1..4295: mol_type = other DNA
gggagacccaagctggctagcgtttaaacttaagcttggtaccgagctcggatccactagtccagtgtggtggaattcagaataaactagtattcttctggtccccacagactcagagagaacccgccaccatgttcgtttttttagttttattacctttagtgagcagccagtgcgtgaacctgatcacccggacccagagctacaccaacagcttcacccggggcgtgtactaccccgacaaggtgttccggagcagcgtgctgcacagcacccaggacctgttcctgcccttcttcagcaacgtgacctggttccacgccatccacgtgagcggcaccaacggcaccaagcggttcgacaaccccgccctgcccttcaacgacggcgtgtacttcgccagcaccgagaagagcaacatcatccggggctggatcttcggcaccaccctggacagcaagacccagagcctgctgatcgtgaacaacgccaccaacgtggtgatcaaggtgtgcgagttccagttctgcaacgaccccttcctggacgtgtaccagaagaacaacaagagctggatggagagcgagttccgggtgtacagcagcgccaacaactgcaccttcgagtacgtgagccagcccttcctgatggacctggagggcaaggagggcaacttcaagaacctgcgggagttcgtgttcaagaacatcgacggctacttcaagatctacagcaagcacacccccatcaacctggagcgggacctgccccagggcttcagcgccctggagcccctggtggacctgcccatcggcatcaacatcacccggttccagaccctgctggccctgcaccggagctacctgacccccgtggacagcagcagcggctggaccgccggcgccgccgcctactacgtgggctacctgcagccccggaccttcctgctgaagtacaacgagaacggcaccatcaccgacgccgtggactgcgccctggaccccctgagcgagaccaagtgcaccctgaagagcttcaccgtggagaagggcatctaccagaccagcaacttccgggtgcagcccaccgagagcatcgtgcgcttccccaacatcaccaacctgtgccccttccacgaggtgttcaacgccaccaccttcgccagcgtgtacgcctggaaccggaagcgcatcagcaactgcgtggccgactacagcgtgatctacaacttcgcccccttcttcgccttcaagtgctacggcgtgagccccaccaagctgaacgacctgtgcttcaccaacgtgtacgccgacagcttcgtgatccggggcaacgaggtgagccagatcgcccccggccagaccggcaacatcgccgactacaactacaagctgcccgacgacttcaccggctgcgtgatcgcctggaacagcaacaagctggacagcaagcccagcggcaactacaactacctgtaccggctgttccggaagagcaagctgaagcccttcgagcgggacatcagcaccgagatctaccaggccggcaacaagccctgcaacggcgtggccggcagcaactgctacagccccctgcggagctacggcttccggcccacctacggcgtgggccaccagccctaccgggtggtggtgctgagcttcgagctgctgcacgcccccgccaccgtgtgcggccccaagaagagcaccaacctggtgaagaacaagtgcgtgaacttcaacttcaacggcctgaccggcaccggcgtgctgaccgagagcaacaagaagttcctgcccttccagcagttcggccgggacatcgccgacaccaccgacgccgtgcgggacccccagaccctggagatcctggacatcaccccctgcagcttcggcggcgtgagcgtgatcacccccggcaccaacaccagcaaccaggtggccgtgctgtaccagggcgtgaactgcaccgaggtgcccgtggccatccacgccgaccagctgacccccacctggcgggtgtacagcaccggcagcaacgtgttccagacccgggccggctgcctgatcggcgccgagtacgtgaacaacagctacgagtgcgacatccccatcggcgccggcatctgcgccagctaccagacccagaccaagagccaccggcgggcccggagcgtggccagccagagcatcatcgcctacaccatgagcctgggcgccgagaacagcgtggcctacagcaacaacagcatcgccatccccaccaacttcaccatcagcgtgaccaccgagatcctgcccgtgagcatgaccaagaccagcgtggactgcaccatgtacatctgcggcgacagcaccgagtgcagcaacctgctgctgcagtacggcagcttctgcacccagctgaagcgggccctgaccggcatcgccgtggagcaggacaagaacacccaggaggtgttcgcccaggtgaagcagatctacaagaccccccccatcaagtacttcggcggcttcaacttcagccagatcctgcccgaccccagcaagcccagcaagcggagcttcatcgaggacctgctgttcaacaaggtgaccctggccgacgccggcttcatcaagcagtacggcgactgcctgggcgacatcgccgcccgggacctgatctgcgcccagaagttcaacggcctgaccgtgctgccccccctgctgaccgacgagatgatcgcccagtacaccagcgccctgctggccggcaccatcaccagcggctggaccttcggcgccggcgccgccctgcagatccccttcgccatgcagatggcctaccggttcaacggcatcggcgtgacccagaacgtgctgtacgagaaccagaagctgatcgccaaccagttcaacagcgccatcggcaagatccaggacagcctgagcagcaccgccagcgccctgggcaagctgcaggacgtggtgaaccacaacgcccaggccctgaacaccctggtgaagcagctgagcagcaagttcggcgccatcagcagcgtgctgaacgacatcctgagccggctggacccccccgaggccgaggtgcagatcgaccggctgatcaccggccggctgcagagcctgcagacctacgtgacccagcagctgatccgggccgccgagatccgggccagcgccaacctggccgccaccaagatgagcgagtgcgtgctgggccagagcaagcgggtggacttctgcggcaagggctaccacctgatgagcttcccccagagcgccccccacggcgtggtgttcctgcacgtgacctacgtgcccgcccaggagaagaacttcaccaccgcccccgccatctgccacgacggcaaggcccacttcccccgggagggcgtgttcgtgagcaacggcacccactggttcgtgacccagcggaacttctacgagccccagatcatcaccaccgacaacaccttcgtgagcggcaactgcgacgtggtgatcggcatcgtgaacaacaccgtgtacgaccccctgcagcccgagctggacagcttcaaggaggagctggacaagtacttcaagaaccacaccagccccgacgtggacctgggcgacatcagcggcatcaacgccagcgtggtgaacatccagaaggagatcgaccggctgaacgaggtggccaagaacctgaacgagagcctgatcgacctgcaggagctgggcaagtacgagcagtacatcaagtggccctggtacatctggctgggcttcatcgccggcctgatcgccatcgtgatggtgaccatcatgctgtgctgcatgaccagctgctgcagctgcctgaagggctgctgcagctgcggcagctgctgcaagtgatgactcgagctggtactgcatgcacgcaatgctagctgcccctttcccgtcctgggtaccccgagtctcccccgacctcgggtcccaggtatgctcccacctccacctgccccactcaccacctctgctagttccagacacctcccaagcacgcagcaatgcagctcaaaacgcttagcctagccacacccccacgggaaacagcagtgattaacctttagcaataaacgaaagtttaactaagctatactaaccccagggttggtcaatttcgtgccagccacaccctggagctagcaaaaaaaaaaaaaaaaaaaaaaaaaaaaaagcatatgactaaaaaaaaaaaaaaaaaaaaaaaaaaaaaaaaaaaaaaaaaaaaaaaaaaaaaaaaaaaaaaaaaaaaaa

SEQ ID NO: 15 - DNA, 4298 bp, synthetic construct
  source 1..4298: mol_type = other DNA
gggagacccaagctggctagcgtttaaacttaagcttggtaccgagctcggatccactagtccagtgtggtggaattcagaataaactagtattcttctggtccccacagactcagagagaacccgccaccatgttcgtttttttagttttattacctttagtgagcagccagtgcgtgaacctgatcacccggacccagagctacaccaacagcttcacccggggcgtgtactaccccgacaaggtgttccggagcagcgtgctgcacagcacccaggacctgttcctgcccttcttcagcaacgtgacctggttccacgccatccacgtgagcggcaccaacggcaccaagcggttcgacaaccccgtgctgcccttcaacgacggcgtgtacttcgccagcaccgagaagagcaacatcatccggggctggatcttcggcaccaccctggacagcaagacccagagcctgctgatcgtgaacaacgccaccaacgtggtgatcaaggtgtgcgagttccagttctgcaacgaccccttcctggacgtgtactaccacgagaacaacaagagccggatggagagcgagctgcgggtgtacagcagcgccaacaactgcaccttcgagtacgtgagccagcccttcctgatggacctggagggcaagcagggcaacttcaagaacctgcgggagttcgtgttcaagaacatcgacggctacttcaagatctacagcaagcacacccccgtgaacctgggccgggacctgccccagggcttcagcgccctggagcccctggtggacctgcccatcggcatcaacatcacccggttccagaccctgctggccctgcaccggagctacctgacccccggcgacagcagcagcagctggaccgccggcgccgccgcctactacgtgggctacctgcagccccggaccttcctgctgaagtacaacgagaacggcaccatcaccgacgccgtggactgcgccctggaccccctgagcgagaccaagtgcaccctgaagagcttcaccgtggagaagggcatctaccagaccagcaacttccgggtgcagcccaccgagagcatcgtgcggttccccaacatcaccaacctgtgccccttccacgaggtgttcaacgccacccggttcgcctccgtgtacgcctggaaccggaagcggatcagcaactgcgtggccgactacagcgtgctgtacaacttcgcccccttcttcgccttcaagtgctacggcgtgagccccaccaagctgaacgacctgtgcttcaccaacgtgtacgccgacagcttcgtgatccggggcaacgaggtgagccagatcgcccccggccagaccggcaacatcgccgactacaactacaagctgcccgacgacttcaccggctgcgtgatcgcctggaacagcaacaagctggacagcaaggtgagcggcaactacaactacctgtaccggctgttccggaagagcaagctgaagcccttcgagcgggacatcagcaccgagatctaccaggccggcaacaagccctgcaacggcgtggccggcttcaactgctacttccccctgcggagctacggcttccggcccacctacggcgtgggccaccagccctaccgggtggtggtgctgagcttcgagctgctgcacgcccccgccaccgtgtgcggccccaagaagagcaccaacctggtgaagaacaagtgcgtgaacttcaacttcaacggcctgaccggcaccggcgtgctgaccgagagcaacaagaagttcctgcccttccagcagttcggccgggacatcgccgacaccaccgacgccgtgcgggacccccagaccctggagatcctggacatcaccccctgcagcttcggcggcgtgagcgtgatcacccccggcaccaacaccagcaaccaggtggccgtgctgtaccagggcgtgaactgcaccgaggtgcccgtggccatccacgccgaccagctgacccccacctggcgggtgtacagcaccggcagcaacgtgttccagacccgggccggctgcctgatcggcgccgagtacgtgaacaacagctacgagtgcgacatccccatcggcgccggcatctgcgccagctaccagacccagaccaagagccaccggcgggcccggagcgtggccagccagagcatcatcgcctacaccatgagcctgggcgccgagaacagcgtggcctacagcaacaacagcatcgccatccccaccaacttcaccatcagcgtgaccaccgagatcctgcccgtgagcatgaccaagaccagcgtggactgcaccatgtacatctgcggcgacagcaccgagtgcagcaacctgctgctgcagtacggcagcttctgcacccagctgaagcgggccctgaccggcatcgccgtggagcaggacaagaacacccaggaggtgttcgcccaggtgaagcagatctacaagaccccccccatcaagtacttcggcggcttcaacttcagccagatcctgcccgaccccagcaagcccagcaagcggagcttcatcgaggacctgctgttcaacaaggtgaccctggccgacgccggcttcatcaagcagtacggcgactgcctgggcgacatcgccgcccgggacctgatctgcgcccagaagttcaacggcctgaccgtgctgccccccctgctgaccgacgagatgatcgcccagtacaccagcgccctgctggccggcaccatcaccagcggctggaccttcggcgccggcgccgccctgcagatccccttcgccatgcagatggcctaccggttcaacggcatcggcgtgacccagaacgtgctgtacgagaaccagaagctgatcgccaaccagttcaacagcgccatcggcaagatccaggacagcctgagcagcaccgccagcgccctgggcaagctgcaggacgtggtgaaccacaacgcccaggccctgaacaccctggtgaagcagctgagcagcaagttcggcgccatcagcagcgtgctgaacgacatcctgagccggctggacccccccgaggccgaggtgcagatcgaccggctgatcaccggccggctgcagagcctgcagacctacgtgacccagcagctgatccgggccgccgagatccgggccagcgccaacctggccgccaccaagatgagcgagtgcgtgctgggccagagcaagcgggtggacttctgcggcaagggctaccacctgatgagcttcccccagagcgccccccacggcgtggtgttcctgcacgtgacctacgtgcccgcccaggagaagaacttcaccaccgcccccgccatctgccacgacggcaaggcccacttcccccgggagggcgtgttcgtgagcaacggcacccactggttcgtgacccagcggaacttctacgagccccagatcatcaccaccgacaacaccttcgtgagcggcaactgcgacgtggtgatcggcatcgtgaacaacaccgtgtacgaccccctgcagcccgagctggacagcttcaaggaggagctggacaagtacttcaagaaccacaccagccccgacgtggacctgggcgacatctccggcatcaacgccagcgtggtgaacatccagaaggagatcgaccggctgaacgaggtggccaagaacctgaacgagagcctgatcgacctgcaggagctgggcaagtacgagcagtacatcaagtggccctggtacatctggctgggcttcatcgccggcctgatcgccatcgtgatggtgaccatcatgctgtgctgcatgaccagctgctgcagctgcctgaagggctgctgcagctgcggcagctgctgcaagtgatgactcgagctggtactgcatgcacgcaatgctagctgcccctttcccgtcctgggtaccccgagtctcccccgacctcgggtcccaggtatgctcccacctccacctgccccactcaccacctctgctagttccagacacctcccaagcacgcagcaatgcagctcaaaacgcttagcctagccacacccccacgggaaacagcagtgattaacctttagcaataaacgaaagtttaactaagctatactaaccccagggttggtcaatttcgtgccagccacaccctggagctagcaaaaaaaaaaaaaaaaaaaaaaaaaaaaaagcatatgactaaaaaaaaaaaaaaaaaaaaaaaaaaaaaaaaaaaaaaaaaaaaaaaaaaaaaaaaaaaaaaaaaaaaaa

SEQ ID NO: 16 - DNA, 4298 bp, synthetic construct
  source 1..4298: mol_type = other DNA
gggagacccaagctggctagcgtttaaacttaagcttggtaccgagctcggatccactagtccagtgtggtggaattcagaataaactagtattcttctggtccccacagactcagagagaacccgccaccatgttcgtttttttagttttattaccattagtgagcagccagtgcgtgaacctgatcacccggacccagagctacaccaacagcttcacccggggcgtgtactaccccgacaaggtgttccggagcagcgtgctgcacagcacccaggacctgttcctgcccttcttcagcaacgtgacctggttccacgccatccacgtgagcggcaccaacggcaccaagcggttcgacaaccccgtgctgcccttcaacgacggcgtgtacttcgccagcaccgagaagagcaacatcatccggggctggatcttcggcaccaccctggacagcaagacccagagcctgctgatcgtgaacaacgccaccaacgtggtgatcaaggtgtgcgagttccagttctgcaacgaccccttcctggacgtgtactaccacgagaacaacaagagccggatggagagcgagctgcgggtgtacagcagcgccaacaactgcaccttcgagtacgtgagccagcccttcctgatggacctggagggcaagcagggcaacttcaagaacctgcgggagttcgtgttcaagaacatcgacggctacttcaagatctacagcaagcacacccccgtgaacctgggccgggacctgccccagggcttcagcgccctggagcccctggtggacctgcccatcggcatcaacatcacccggttccagaccctgctggccctgcaccggagctacctgacccccggcgacagcagcagcagctggaccgccggcgccgccgcctactacgtgggctacctgcagccccggaccttcctgctgaagtacaacgagaacggcaccatcaccgacgccgtggactgcgccctggaccccctgagcgagaccaagtgcaccctgaagagcttcaccgtggagaagggcatctaccagaccagcaacttccgggtgcagcccaccgagagcatcgtgcggttccccaacatcaccaacctgtgccccttccacgaggtgttcaacgccacccggttcgccagcgtgtacgcctggaaccggaagcggatcagcaactgcgtggccgactacagcgtgctgtacaacttcgcccccttcttcgccttcaagtgctacggcgtgagccccaccaagctgaacgacctgtgcttcaccaacgtgtacgccgacagcttcgtgatccggggcaacgaggtgagccagatcgcccccggccagaccggcaacatcgccgactacaactacaagctgcccgacgacttcaccggctgcgtgatcgcctggaacagcaacaagctggacagcaaggtgagcggcaactacaactacctgtaccggctgttccggaagagcaagctgaagcccttcgagcgggacatcagcaccgagatctaccaggccggcaacaagccctgcaacggcgtggccggcttcaactgctacttccccctgcggagctacggcttccggcccacctacggcgtgggccaccagccctaccgggtggtggtgctgagcttcgagctgctgcacgcccccgccaccgtgtgcggccccaagaagagcaccaacctggtgaagaacaagtgcgtgaacttcaacttcaacggcctgaccggcaccggcgtgctgaccgagagcaacaagaagttcctgcccttccagcagttcggccgggacatcgccgacaccaccgacgccgtgcgggacccccagaccctggagatcctggacatcaccccctgcagcttcggcggcgtgagcgtgatcacccccggcaccaacaccagcaaccaggtggccgtgctgtaccagggcgtgaactgcaccgaggtgcccgtggccatccacgccgaccagctgacccccacctggcgggtgtacagcaccggcagcaacgtgttccagacccgggccggctgcctgatcggcgccgagtacgtgaacaacagctacgagtgcgacatccccatcggcgccggcatctgcgccagctaccagacccagaccaagagccaccggcgggcccggagcgtggccagccagagcatcatcgcctacaccatgagcctgggcgccgagaacagcgtggcctacagcaacaacagcatcgccatccccaccaacttcaccatcagcgtgaccaccgagatcctgcccgtgagcatgaccaagaccagcgtggactgcaccatgtacatctgcggcgacagcaccgagtgcagcaacctgctgctgcagtacggcagcttctgcacccagctgaagcgggccctgaccggcatcgccgtggagcaggacaagaacacccaggaggtgttcgcccaggtgaagcagatctacaagaccccccccatcaagtacttcggcggcttcaacttcagccagatcctgcccgaccccagcaagcccagcaagcggagcttcatcgaggacctgctgttcaacaaggtgaccctggccgacgccggcttcatcaagcagtacggcgactgcctgggcgacatcgccgcccgggacctgatctgcgcccagaagttcaacggcctgaccgtgctgccccccctgctgaccgacgagatgatcgcccagtacaccagcgccctgctggccggcaccatcaccagcggctggaccttcggcgccggcgccgccctgcagatccccttcgccatgcagatggcctaccggttcaacggcatcggcgtgacccagaacgtgctgtacgagaaccagaagctgatcgccaaccagttcaacagcgccatcggcaagatccaggacagcctgagcagcaccgccagcgccctgggcaagctgcaggacgtggtgaaccacaacgcccaggccctgaacaccctggtgaagcagctgagcagcaagttcggcgccatcagcagcgtgctgaacgacatcctgagccggctggacccccccgaggccgaggtgcagatcgaccggctgatcaccggccggctgcagagcctgcagacctacgtgacccagcagctgatccgggccgccgagatccgggccagcgccaacctggccgccaccaagatgagcgagtgcgtgctgggccagagcaagcgggtggacttctgcggcaagggctaccacctgatgtccttcccccagagcgccccccacggcgtggtgttcctgcacgtgacctacgtgcccgcccaggagaagaacttcaccaccgcccccgccatctgccacgacggcaaggcccacttcccccgggagggcgtgttcgtgagcaacggcacccactggttcgtgacccagcggaacttctacgagccccagatcatcaccaccgacaacaccttcgtgagcggcaactgcgacgtggtgatcggcatcgtgaacaacaccgtgtacgaccccctgcagcccgagctggacagcttcaaggaggagctggacaagtacttcaagaaccacaccagccccgacgtggacctgggcgacatcagcggcatcaacgccagcgtggtgaacatccagaaggagatcgaccggctgaacgaggtggccaagaacctgaacgagagcctgatcgacctgcaggagctgggcaagtacgagcagtacatcaagtggccctggtacatctggctgggcttcatcgccggcctgatcgccatcgtgatggtgaccatcatgctgtgctgcatgaccagctgctgcagctgcctgaagggctgctgcagctgcggcagctgctgcaagtgatgactcgagctggtactgcatgcacgcaatgctagctgcccctttcccgtcctgggtaccccgagtctcccccgacctcgggtcccaggtatgctcccacctccacctgccccactcaccacctctgctagttccagacacctcccaagcacgcagcaatgcagctcaaaacgcttagcctagccacacccccacgggaaacagcagtgattaacctttagcaataaacgaaagtttaactaagctatactaaccccagggttggtcaatttcgtgccagccacaccctggagctagcaaaaaaaaaaaaaaaaaaaaaaaaaaaaaagcatatgactaaaaaaaaaaaaaaaaaaaaaaaaaaaaaaaaaaaaaaaaaaaaaaaaaaaaaaaaaaaaaaaaaaaaaa

SEQ ID NO: 17 - DNA, 4343 bp, synthetic construct
  source 1..4343: mol_type = other DNA
gggagacccaagctggctagcgtttaaacttaagcttggtaccgagctcggatccactagtccagtgtggtggaattcagaataaactagtattcttctggtccccacagactcagagagaacccgccaccatgttcgtttttttagttttattacctttagtgagcagccagtgcgtgaacctgatcacccggacccagagctacaccaacagcttcacccggggcgtgtactaccccgacaaggtgttccggagcagcgtgctgcacagcacccaggacctgttcctgcccttcttcagcaacgtgacctggttccacgccatcagcggcaccaacggcaccaagcggttcgacaaccccgtgctgcccttcaacgacggcgtgtacttcgccagcaccgagaagagcaacatcatccggggctggatcttcggcaccaccctggacagcaagacccagagcctgctgatcgtgaacaacgccaccaacgtggtgatcaaggtgtgcgagttccagttctgcaacgaccccttcctggacgtgtaccacaagaacaacaagtcctggatggagagcgagttccgggtgtacagcagcgccaacaactgcaccttcgagtacgtgagccagcccttcctgatggacctggagggcaagcagggcaacttcaagaacctgcgggagttcgtgttcaagaacatcgacggctacttcaagatctacagcaagcacacccccatcaacctgggccgggacctgccccagggcttcagcgccctggagcccctggtggacctgcccatcggcatcaacatcacccggttccagaccctgctggccctgcaccggagctacctgacccccggcgacagcagcagcggctggaccgccggcgccgccgcctactacgtgggctacctgcagccccggaccttcctgctgaagtacaacgagaacggcaccatcaccgacgccgtggactgcgccctggaccccctgagcgagaccaagtgcaccctgaagagcttcaccgtggagaagggcatctaccagaccagcaacttccgggtgcagcccaccgagagcatcgtgcggttccccaacatcaccaacctgtgccccttcgacgaggtgttcaacgccacccggttcgccagcgtgtacgcctggaaccggaagcggatcagcaactgcgtggccgactacagcgtgctgtacaacttcgcccccttcttcgccttcaagtgctacggcgtgagccccaccaagctgaacgacctgtgcttcaccaacgtgtacgccgacagcttcgtgatccggggcaacgaggtgagccagatcgcccccggccagaccggcaacatcgccgactacaactacaagctgcccgacgacttcaccggctgcgtgatcgcctggaacagcaacaagctggacagcaccgtgggcggcaactacaactaccggtaccggctgttccggaagagcaagctgaagcccttcgagcgggacatcagcaccgagatctaccaggccggcaacaagccctgcaacggcgtggccggcgtgaactgctacttccccctgcagagctacggcttccggcccacctacggcgtgggccaccagccctaccgggtggtggtgctgagcttcgagctgctgcacgcccccgccaccgtgtgcggccccaagaagagcaccaacctggtgaagaacaagtgcgtgaacttcaacttcaacggcctgaccggcaccggcgtgctgaccgagagcaacaagaagttcctgcccttccagcagttcggccgggacatcgccgacaccaccgacgccgtgcgggacccccagaccctggagatcctggacatcaccccctgcagcttcggcggcgtgtccgtgatcacccccggcaccaacaccagcaaccaggtggccgtgctgtaccagggcgtgaactgcaccgaggtgcccgtggccatccacgccgaccagctgacccccacctggcgggtgtacagcaccggcagcaacgtgttccagacccgggccggctgcctgatcggcgccgagtacgtgaacaacagctacgagtgcgacatccccatcggcgccggcatctgcgccagctaccagacccagaccaagagccaccggcgggcccggagcgtggccagccagagcatcatcgcctacaccatgagcctgggcgccgagaacagcgtggcctacagcaacaacagcatcgccatccccaccaacttcaccatcagcgtgaccaccgagatcctgcccgtgagcatgaccaagaccagcgtggactgcaccatgtacatctgcggcgacagcaccgagtgcagcaacctgctgctgcagtacggcagcttctgcacccagctgaagcgggccctgaccggcatcgccgtggagcaggacaagaacacccaggaggtgttcgcccaggtgaagcagatctacaagaccccccccatcaagtacttcggcggcttcaacttcagccagatcctgcccgaccccagcaagcccagcaagcggagcttcatcgaggacctgctgttcaacaaggtgaccctggccgacgccggcttcatcaagcagtacggcgactgcctgggcgacatcgccgcccgggacctgatctgcgcccagaagttcaacggcctgaccgtgctgccccccctgctgaccgacgagatgatcgcccagtacaccagcgccctgctggccggcaccatcaccagcggctggaccttcggcgccggcgccgccctgcagatccccttcgccatgcagatggcctaccggttcaacggcatcggcgtgacccagaacgtgctgtacgagaaccagaagctgatcgccaaccagttcaacagcgccatcggcaagatccaggacagcctgagcagcaccgccagcgccctgggcaagctgcaggacgtggtgaaccacaacgcccaggccctgaacaccctggtgaagcagctgagcagcaagttcggcgccatcagcagcgtgctgaacgacatcctgagccggctggacccccccgaggccgaggtgcagatcgaccggctgatcaccggccggctgcagagcctgcagacctacgtgacccagcagctgatccgggccgccgagatccgggccagcgccaacctggccgccaccaagatgagcgagtgcgtgctgggccagagcaagcgggtggacttctgcggcaagggctaccacctgatgagcttcccccagagcgccccccacggcgtggtgttcctgcacgtgacctacgtgcccgcccaggagaagaacttcaccaccgcccccgccatctgccacgacggcaaggcccacttcccccgggagggcgtgttcgtgagcaacggcacccactggttcgtgacccagcggaacttctacgagccccagatcatcaccaccgacaacaccttcgtgagcggcaactgcgacgtggtgatcggcatcgtgaacaacaccgtgtacgaccccctgcagcccgagctggacagcttcaaggaggagctggacaagtacttcaagaaccacaccagccccgacgtggacctgggcgacatcagcggcatcaacgccagcgtggtgaacatccagaaggagatcgaccggctgaacgaggtggccaagaacctgaacgagagcctgatcgacctgcaggagctgggcaagtacgagcagtacatcaagtggccctggtacatctggctgggcttcatcgccggcctgatcgccatcgtgatggtgaccatcatgctgtgctgcatgaccagctgctgcagctgcctgaagggctgctgcagctgcggcagctgctgcaagttcgacgaggacgacagcgagcccgtgctgaagggcgtgaagctgcactacacctgatgactcgagctggtactgcatgcacgcaatgctagctgcccctttcccgtcctgggtaccccgagtctcccccgacctcgggtcccaggtatgctcccacctccacctgccccactcaccacctctgctagttccagacacctcccaagcacgcagcaatgcagctcaaaacgcttagcctagccacacccccacgggaaacagcagtgattaacctttagcaataaacgaaagtttaactaagctatactaaccccagggttggtcaatttcgtgccagccacaccctggagctagcaaaaaaaaaaaaaaaaaaaaaaaaaaaaaagcatatgactaaaaaaaaaaaaaaaaaaaaaaaaaaaaaaaaaaaaaaaaaaaaaaaaaaaaaaaaaaaaaaaaaaaaaa

SEQ ID NO: 18 - DNA, 4343 bp, synthetic construct
  source 1..4343: mol_type = other DNA
gggagacccaagctggctagcgtttaaacttaagcttggtaccgagctcggatccactagtccagtgtggtggaattcagaataaactagtattcttctggtccccacagactcagagagaacccgccaccatgttcgtttttttagttttattaccattagtgagcagccagtgcgtgaacctgatcacccggacccagagctacaccaacagcttcacccggggcgtgtactaccccgacaaggtgttccggagcagcgtgctgcacagcacccaggacctgttcctgcccttcttcagcaacgtgacctggttccacgccatcagcggcaccaacggcaccaagcggttcgacaaccccgtgctgcccttcaacgacggcgtgtacttcgccagcaccgagaagagcaacatcatccggggctggatcttcggcaccaccctggacagcaagacccagagcctgctgatcgtgaacaacgccaccaacgtggtgatcaaggtgtgcgagttccagttctgcaacgaccccttcctggacgtgtaccacaagaacaacaagagctggatggagagcgagttccgggtgtacagcagcgccaacaactgcaccttcgagtacgtgagccagcccttcctgatggacctggagggcaagcagggcaacttcaagaacctgcgggagttcgtgttcaagaacatcgacggctacttcaagatctacagcaagcacacccccatcaacctgggccgggacctgccccagggcttcagcgcgctggagcccctggtggacctgcccatcggcatcaacatcacccggttccagaccctgctggccctgcaccggagctacctgacccccggcgacagcagcagcggctggaccgccggcgccgccgcctactacgtgggctacctgcagccccggaccttcctgctgaagtacaacgagaacggcaccatcaccgacgccgtggactgcgccctggaccccctgagcgagaccaagtgcaccctgaagagcttcaccgtggagaagggcatctaccagaccagcaacttccgggtgcagcccaccgagagcatcgtgcggttccccaacatcaccaacctgtgccccttcgacgaggtgttcaacgccacccggttcgccagcgtgtacgcctggaaccggaagcggatcagcaactgcgtggccgactacagcgtgctgtacaacttcgcccccttcttcgccttcaagtgctacggcgtgagccccaccaagctgaacgacctgtgcttcaccaacgtgtacgccgacagcttcgtgatccggggcaacgaggtgagccagatcgcccccggccagaccggcaacatcgccgactacaactacaagctgcccgacgacttcaccggctgcgtgatcgcctggaacagcaacaagctggacagcaccgtgggcggcaactacaactaccggtaccggctgttccggaagagcaagctgaagcccttcgagcgggacatcagcaccgagatctaccaggccggcaacaagccctgcaacggcgtggccggcgtgaactgctacttccccctgcagagctacggcttccggcccacctacggcgtgggccaccagccctaccgggtggtggtgctgagcttcgagctgctgcacgcccccgccaccgtgtgcggccccaagaagagcaccaacctggtgaagaacaagtgcgtgaacttcaacttcaacggcctgaccggcaccggcgtgctgaccgagagcaacaagaagttcctgcccttccagcagttcggccgggacatcgccgacaccaccgacgccgtgcgggacccccagaccctggagatcctggacatcaccccctgcagcttcggcggcgtgagcgtgatcacccccggcaccaacaccagcaaccaggtggccgtgctgtaccagggcgtgaactgcaccgaggtgcccgtggccatccacgccgaccagctgacccccacctggcgggtgtacagcaccggcagcaacgtgttccagacccgggccggctgcctgatcggcgccgagtacgtgaacaacagctacgagtgcgacatccccatcggcgccggcatctgcgccagctaccagacccagaccaagagccaccggcgggcccggagcgtggccagccagagcatcatcgcctacaccatgagcctgggcgccgagaacagcgtggcctacagcaacaacagcatcgccatccccaccaacttcaccatctccgtgaccaccgagatcctgcccgtgagcatgaccaagaccagcgtggactgcaccatgtacatctgcggcgacagcaccgagtgcagcaacctgctgctgcagtacggcagcttctgcacccagctgaagcgggccctgaccggcatcgccgtggagcaggacaagaacacccaggaggtgttcgcccaggtgaagcagatctacaagaccccccccatcaagtacttcggcggcttcaacttcagccagatcctgcccgaccccagcaagcccagcaagcggagcttcatcgaggacctgctgttcaacaaggtgaccctggccgacgccggcttcatcaagcagtacggcgactgcctgggcgacatcgccgcccgggacctgatctgcgcccagaagttcaacggcctgaccgtgctgccccccctgctgaccgacgagatgatcgcccagtacaccagcgccctgctggccggcaccatcaccagcggctggaccttcggcgccggcgccgccctgcagatccccttcgccatgcagatggcctaccggttcaacggcatcggcgtgacccagaacgtgctgtacgagaaccagaagctgatcgccaaccagttcaacagcgccatcggcaagatccaggacagcctgagcagcaccgccagcgccctgggcaagctgcaggacgtggtgaaccacaacgcccaggccctgaacaccctggtgaagcagctgagcagcaagttcggcgccatcagcagcgtgctgaacgacatcctgagccggctggacccccccgaggccgaggtgcagatcgaccggctgatcaccggccggctgcagagcctgcagacctacgtgacccagcagctgatccgggccgccgagatccgggccagcgccaacctggccgccaccaagatgagcgagtgcgtgctgggccagagcaagcgggtggacttctgcggcaagggctaccacctgatgagcttcccccagagcgccccccacggcgtggtgttcctgcacgtgacctacgtgcccgcccaggagaagaacttcaccaccgcccccgccatctgccacgacggcaaggcccacttcccccgggagggcgtgttcgtgagcaacggcacccactggttcgtgacccagcggaacttctacgagccccagatcatcaccaccgacaacaccttcgtgagcggcaactgcgacgtggtgatcggcatcgtgaacaacaccgtgtacgaccccctgcagcccgagctggacagcttcaaggaggagctggacaagtacttcaagaaccacaccagccccgacgtggacctgggcgacatcagcggcatcaacgccagcgtggtgaacatccagaaggagatcgaccggctgaacgaggtggccaagaacctgaacgagagcctgatcgacctgcaggagctgggcaagtacgagcagtacatcaagtggccctggtacatctggctgggcttcatcgccggcctgatcgccatcgtgatggtgaccatcatgctgtgctgcatgaccagctgctgcagctgcctgaagggctgctgcagctgcggcagctgctgcaagttcgacgaggacgacagcgagcccgtgctgaagggcgtgaagctgcactacacctgatgactcgagctggtactgcatgcacgcaatgctagctgcccctttcccgtcctgggtaccccgagtctcccccgacctcgggtcccaggtatgctcccacctccacctgccccactcaccacctctgctagttccagacacctcccaagcacgcagcaatgcagctcaaaacgcttagcctagccacacccccacgggaaacagcagtgattaacctttagcaataaacgaaagtttaactaagctatactaaccccagggttggtcaatttcgtgccagccacaccctggagctagcaaaaaaaaaaaaaaaaaaaaaaaaaaaaaagcatatgactaaaaaaaaaaaaaaaaaaaaaaaaaaaaaaaaaaaaaaaaaaaaaaaaaaaaaaaaaaaaaaaaaaaaaa

SEQ ID NO: 19 - DNA, 4346 bp, synthetic construct
  source 1..4346: mol_type = other DNA
gggagacccaagctggctagcgtttaaacttaagcttggtaccgagctcggatccactagtccagtgtggtggaattcagaataaactagtattcttctggtccccacagactcagagagaacccgccaccatgttcgtttttttagttttattacctttagtgagcagccagtgcgtgaacctgatcacccggacccagagctacaccaacagcttcacccggggcgtgtactaccccgacaaggtgttccggagcagcgtgctgcacagcacccaggacctgttcctgcccttcttcagcaacgtgacctggttccacgccatcagcggcaccaacggcaccaagcggttcgacaaccccgtgctgcccttcaacgacggcgtgtacttcgccagcaccgagaagagcaacatcatccggggctggatcttcggcaccaccctggacagcaagacccagagcctgctgatcgtgaacaacgccaccaacgtggtgatcaaggtgtgcgagttccagttctgcaacgaccccttcctggacgtgtactaccacaagaacaacaagtcctggatggagagcgagttccgggtgtacagcagcgccaacaactgcaccttcgagtacgtgagccagcccttcctgatggacctggagggcaagcagggcaacttcaagaacctgcgggagttcgtgttcaagaacatcgacggctacttcaagatctacagcaagcacacccccatcaacctgggccgggacctgccccagggcttcagcgccctggagcccctggtggacctgcccatcggcatcaacatcacccggttccagaccctgctggccctgcaccggagctacctgacccccggcgacagcagcagcggctggaccgccggcgccgccgcctactacgtgggctacctgcagccccggaccttcctgctgaagtacaacgagaacggcaccatcaccgacgccgtggactgcgccctggaccccctgagcgagaccaagtgcaccctgaagagcttcaccgtggagaagggcatctaccagaccagcaacttccgggtgcagcccaccgagagcatcgtgcggttccccaacatcaccaacctgtgccccttcgacgaggtgttcaacgccaccaccttcgccagcgtgtacgcctggaaccggaagcggatcagcaactgcgtggccgactacagcgtgctgtacaacttcgcccccttcttcgccttcaagtgctacggcgtgagccccaccaagctgaacgacctgtgcttcaccaacgtgtacgccgacagcttcgtgatccggggcaacgaggtgagccagatcgcccccggccagaccggcaacatcgccgactacaactacaagctgcccgacgacttcaccggctgcgtgatcgcctggaacagcaacaagctggacagcaaggtgggcggcaactacaactaccggtaccggctgttccggaagagcaacctgaagcccttcgagcgggacatcagcaccgagatctaccaggccggcaacaagccctgcaacggcgtggccggcgtgaactgctacttccccctgcagagctacggcttccggcccacctacggcgtgggccaccagccctaccgggtggtggtgctgagcttcgagctgctgcacgcccccgccaccgtgtgcggccccaagaagagcaccaacctggtgaagaacaagtgcgtgaacttcaacttcaacggcctgaccggcaccggcgtgctgaccgagagcaacaagaagttcctgcccttccagcagttcggccgggacatcgccgacaccaccgacgccgtgcgggacccccagaccctggagatcctggacatcaccccctgcagcttcggcggcgtgtccgtgatcacccccggcaccaacaccagcaaccaggtggccgtgctgtaccagggcgtgaactgcaccgaggtgcccgtggccatccacgccgaccagctgacccccacctggcgggtgtacagcaccggcagcaacgtgttccagacccgggccggctgcctgatcggcgccgagtacgtgaacaacagctacgagtgcgacatccccatcggcgccggcatctgcgccagctaccagacccagaccaagagccaccggcgggcccggagcgtggccagccagagcatcatcgcctacaccatgagcctgggcgccgagaacagcgtggcctacagcaacaacagcatcgccatccccaccaacttcaccatcagcgtgaccaccgagatcctgcccgtgagcatgaccaagaccagcgtggactgcaccatgtacatctgcggcgacagcaccgagtgcagcaacctgctgctgcagtacggcagcttctgcacccagctgaagcgggccctgaccggcatcgccgtggagcaggacaagaacacccaggaggtgttcgcccaggtgaagcagatctacaagaccccccccatcaagtacttcggcggcttcaacttcagccagatcctgcccgaccccagcaagcccagcaagcggagcttcatcgaggacctgctgttcaacaaggtgaccctggccgacgccggcttcatcaagcagtacggcgactgcctgggcgacatcgccgcccgggacctgatctgcgcccagaagttcaacggcctgaccgtgctgccccccctgctgaccgacgagatgatcgcccagtacaccagcgccctgctggccggcaccatcaccagcggctggaccttcggcgccggcgccgccctgcagatccccttcgccatgcagatggcctaccggttcaacggcatcggcgtgacccagaacgtgctgtacgagaaccagaagctgatcgccaaccagttcaacagcgccatcggcaagatccaggacagcctgagcagcaccgccagcgccctgggcaagctgcaggacgtggtgaaccacaacgcccaggccctgaacaccctggtgaagcagctgagcagcaagttcggcgccatcagcagcgtgctgaacgacatcctgagccggctggacccccccgaggccgaggtgcagatcgaccggctgatcaccggccggctgcagagcctgcagacctacgtgacccagcagctgatccgggccgccgagatccgggccagcgccaacctggccgccaccaagatgagcgagtgcgtgctgggccagagcaagcgggtggacttctgcggcaagggctaccacctgatgagcttcccccagagcgccccccacggcgtggtgttcctgcacgtgacctacgtgcccgcccaggagaagaacttcaccaccgcccccgccatctgccacgacggcaaggcccacttcccccgggagggcgtgttcgtgagcaacggcacccactggttcgtgacccagcggaacttctacgagccccagatcatcaccaccgacaacaccttcgtgagcggcaactgcgacgtggtgatcggcatcgtgaacaacaccgtgtacgaccccctgcagcccgagctggacagcttcaaggaggagctggacaagtacttcaagaaccacaccagccccgacgtggacctgggcgacatcagcggcatcaacgccagcgtggtgaacatccagaaggagatcgaccggctgaacgaggtggccaagaacctgaacgagagcctgatcgacctgcaggagctgggcaagtacgagcagtacatcaagtggccctggtacatctggctgggcttcatcgccggcctgatcgccatcgtgatggtgaccatcatgctgtgctgcatgaccagctgctgcagctgcctgaagggctgctgcagctgcggcagctgctgcaagttcgacgaggacgacagcgagcccgtgctgaagggcgtgaagctgcactacacctgatgactcgagctggtactgcatgcacgcaatgctagctgcccctttcccgtcctgggtaccccgagtctcccccgacctcgggtcccaggtatgctcccacctccacctgccccactcaccacctctgctagttccagacacctcccaagcacgcagcaatgcagctcaaaacgcttagcctagccacacccccacgggaaacagcagtgattaacctttagcaataaacgaaagtttaactaagctatactaaccccagggttggtcaatttcgtgccagccacaccctggagctagcaaaaaaaaaaaaaaaaaaaaaaaaaaaaaagcatatgactaaaaaaaaaaaaaaaaaaaaaaaaaaaaaaaaaaaaaaaaaaaaaaaaaaaaaaaaaaaaaaaaaaaaaa

SEQ ID NO: 20 - DNA, 4346 bp, synthetic construct
  source 1..4346: mol_type = other DNA
gggagacccaagctggctagcgtttaaacttaagcttggtaccgagctcggatccactagtccagtgtggtggaattcagaataaactagtattcttctggtccccacagactcagagagaacccgccaccatgttcgtttttttagttttattaccattagtgagcagccagtgcgtgaacctgatcacccggacccagagctacaccaacagcttcacccggggcgtgtactaccccgacaaggtgttccggagcagcgtgctgcacagcacccaggacctgttcctgcccttcttcagcaacgtgacctggttccacgccatcagcggcaccaacggcaccaagcggttcgacaaccccgtgctgcccttcaacgacggcgtgtacttcgccagcaccgagaagagcaacatcatccggggctggatcttcggcaccaccctggacagcaagacccagagcctgctgatcgtgaacaacgccaccaacgtggtgatcaaggtgtgcgagttccagttctgcaacgaccccttcctggacgtgtactaccacaagaacaacaagagctggatggagagcgagttccgggtgtacagcagcgccaacaactgcaccttcgagtacgtgagccagcccttcctgatggacctggagggcaagcagggcaacttcaagaacctgcgggagttcgtgttcaagaacatcgacggctacttcaagatctacagcaagcacacccccatcaacctgggccgggacctgccccagggcttcagcgccctggagcccctggtggacctgcccatcggcatcaacatcacccggttccagaccctgctggccctgcaccggagctacctgacccccggcgacagcagcagcggctggaccgccggcgccgccgcctactacgtgggctacctgcagccccggaccttcctgctgaagtacaacgagaacggcaccatcaccgacgccgtggactgcgccctggaccccctgagcgagaccaagtgcaccctgaagagcttcaccgtggagaagggcatctaccagaccagcaacttccgggtgcagcccaccgagagcatcgtgcggttccccaacatcaccaacctgtgccccttcgacgaggtgttcaacgccaccaccttcgccagcgtgtacgcctggaaccggaagcggatcagcaactgcgtggccgactacagcgtgctgtacaacttcgcccccttcttcgccttcaagtgctacggcgtgagccccaccaagctgaacgacctgtgcttcaccaacgtgtacgccgacagcttcgtgatccggggcaacgaggtgagccagatcgcccccggccagaccggcaacatcgccgactacaactacaagctgcccgacgacttcaccggctgcgtgatcgcctggaacagcaacaagctggacagcaaggtgggcggcaactacaactaccggtaccggctgttccggaagagcaacctgaagcccttcgagcgggacatcagcaccgagatctaccaggccggcaacaagccctgcaacggcgtggccggcgtgaactgctacttccccctgcagagctacggcttccggcccacctacggcgtgggccaccagccctaccgggtggtggtgctgagcttcgagctgctgcacgcccccgccaccgtgtgcggccccaagaagagcaccaacctggtgaagaacaagtgcgtgaacttcaacttcaacggcctgaccggcaccggcgtgctgaccgagagcaacaagaagttcctgcccttccagcagttcggccgggacatcgccgacaccaccgacgccgtgcgggacccccagaccctggagatcctggacatcaccccctgcagcttcggcggcgtgagcgtgatcacccccggcaccaacaccagcaaccaggtggccgtgctgtaccagggcgtgaactgcaccgaggtgcccgtggccatccacgccgaccagctgacccccacctggcgggtgtacagcaccggcagcaacgtgttccagacccgggccggctgcctgatcggcgccgagtacgtgaacaacagctacgagtgcgacatccccatcggcgccggcatctgcgccagctaccagacccagaccaagagccaccggcgggcccggagcgtggccagccagagcatcatcgcctacaccatgagcctgggcgccgagaacagcgtggcctacagcaacaacagcatcgccatccccaccaacttcaccatcagcgtgaccaccgagatcctgcccgtgagcatgaccaagaccagcgtggactgcaccatgtacatctgcggcgacagcaccgagtgcagcaacctgctgctgcagtacggcagcttctgcacccagctgaagcgggccctgaccggcatcgccgtggagcaggacaagaacacccaggaggtgttcgcccaggtgaagcagatctacaagaccccccccatcaagtacttcggcggcttcaacttcagccagatcctgcccgaccccagcaagcccagcaagcggagcttcatcgaggacctgctgttcaacaaggtgaccctggccgacgccggcttcatcaagcagtacggcgactgcctgggcgacatcgccgcccgggacctgatctgcgcccagaagttcaacggcctgaccgtgctgccccccctgctgaccgacgagatgatcgcccagtacaccagcgccctgctggccggcaccatcaccagcggctggaccttcggcgccggcgccgccctgcagatccccttcgccatgcagatggcctaccggttcaacggcatcggcgtgacccagaacgtgctgtacgagaaccagaagctgatcgccaaccagttcaacagcgccatcggcaagatccaggacagcctgagcagcaccgccagcgccctgggcaagctgcaggacgtggtgaaccacaacgcccaggccctgaacaccctggtgaagcagctgagcagcaagttcggcgccatcagcagcgtgctgaacgacatcctgagccggctggacccccccgaggccgaggtgcagatcgaccggctgatcaccggccggctgcagagcctgcagacctacgtgacccagcagctgatccgggccgccgagatccgggccagcgccaacctggccgccaccaagatgagcgagtgcgtgctgggccagagcaagcgggtggacttctgcggcaagggctaccacctgatgtccttcccccagagcgccccccacggcgtggtgttcctgcacgtgacctacgtgcccgcccaggagaagaacttcaccaccgcccccgccatctgccacgacggcaaggcccacttcccccgggagggcgtgttcgtgagcaacggcacccactggttcgtgacccagcggaacttctacgagccccagatcatcaccaccgacaacaccttcgtgagcggcaactgcgacgtggtgatcggcatcgtgaacaacaccgtgtacgaccccctgcagcccgagctggacagcttcaaggaggagctggacaagtacttcaagaaccacaccagccccgacgtggacctgggcgacatcagcggcatcaacgccagcgtggtgaacatccagaaggagatcgaccggctgaacgaggtggccaagaacctgaacgagagcctgatcgacctgcaggagctgggcaagtacgagcagtacatcaagtggccctggtacatctggctgggcttcatcgccggcctgatcgccatcgtgatggtgaccatcatgctgtgctgcatgaccagctgctgcagctgcctgaagggctgctgcagctgcggcagctgctgcaagttcgacgaggacgacagcgagcccgtgctgaagggcgtgaagctgcactacacctgatgactcgagctggtactgcatgcacgcaatgctagctgcccctttcccgtcctgggtaccccgagtctcccccgacctcgggtcccaggtatgctcccacctccacctgccccactcaccacctctgctagttccagacacctcccaagcacgcagcaatgcagctcaaaacgcttagcctagccacacccccacgggaaacagcagtgattaacctttagcaataaacgaaagtttaactaagctatactaaccccagggttggtcaatttcgtgccagccacaccctggagctagcaaaaaaaaaaaaaaaaaaaaaaaaaaaaaagcatatgactaaaaaaaaaaaaaaaaaaaaaaaaaaaaaaaaaaaaaaaaaaaaaaaaaaaaaaaaaaaaaaaaaaaaaa

SEQ ID NO: 21 - DNA, 4352 bp, synthetic construct
  source 1..4352: mol_type = other DNA
gggagacccaagctggctagcgtttaaacttaagcttggtaccgagctcggatccactagtccagtgtggtggaattcagaataaactagtattcttctggtccccacagactcagagagaacccgccaccatgttcgtttttttagttttattacctttagtgtccagccagtgcgtgaacctgatcacccggacccagagctacaccaacagcttcacccggggcgtgtactaccccgacaaggtgttccggagcagcgtgctgcacagcacccaggacctgttcctgcccttcttcagcaacgtgacctggttccacgccatccacgtgagcggcaccaacggcaccaagcggttcgacaaccccgtgctgcccttcaacgacggcgtgtacttcgccagcaccgagaagagcaacatcatccggggctggatcttcggcaccaccctggacagcaagacccagagcctgctgatcgtgaacaacgccaccaacgtggtgatcaaggtgtgcgagttccagttctgcaacgaccccttcctggacgtgtactaccacgagaacaacaagagccggatggagagcgagctgcgggtgtacagcagcgccaacaactgcaccttcgagtacgtgagccagcccttcctgatggacctggagggcaagcagggcaacttcaagaacctgcgggagttcgtgttcaagaacatcgacggctacttcaagatctacagcaagcacacccccgtgaacctgggccgggacctgccccagggcttcagcgccctggagcccctggtggacctgcccatcggcatcaacatcacccggttccagaccctgctggccctgcaccggagctacctgacccccggcgacagcagcagcagctggaccgccggcgccgccgcctactacgtgggctacctgcagccccggaccttcctgctgaagtacaacgagaacggcaccatcaccgacgccgtggactgcgccctggaccccctgagcgagaccaagtgcaccctgaagagcttcaccgtggagaagggcatctaccagaccagcaacttccgggtgcagcccaccgagagcatcgtgcggttccccaacatcaccaacctgtgccccttccacgaggtgttcaacgccaccaccttcgccagcgtgtacgcctggaaccggaagcggatcagcaactgcgtggccgactacagcgtgctgtacaacttcgcccccttcttcgccttcaagtgctacggcgtgagccccaccaagctgaacgacctgtgcttcaccaacgtgtacgccgacagcttcgtgatccggggcaacgaggtgagccagatcgcccccggccagaccggcaacatcgccgactacaactacaagctgcccgacgacttcaccggctgcgtgatcgcctggaacagcaacaagctggacagcaccgtgagcggcaactacaactaccggtaccggctgttccggaagagcaagctgaagcccttcgagcgggacatcagcaccgagatctaccaggccggcaacaagccctgcaacggcgtggccggcagcaactgctacttccccctgcagagctacggcttccggcccacctacggcgtgggccaccagccctaccgggtggtggtgctgagcttcgagctgctgcacgcccccgccaccgtgtgcggccccaagaagagcaccaacctggtgaagaacaagtgcgtgaacttcaacttcaacggcctgaccggcaccggcgtgctgaccgagagcaacaagaagttcctgcccttccagcagttcggccgggacatcgccgacaccaccgacgccgtgcgggacccccagaccctggagatcctggacatcaccccctgcagcttcggcggcgtgagcgtgatcacccccggcaccaacaccagcaaccaggtggccgtgctgtaccagggcgtgaactgcaccgaggtgcccgtggccatccacgccgaccagctgacccccacctggcgggtgtacagcaccggcagcaacgtgttccagacccgggccggctgcctgatcggcgccgagtacgtgaacaacagctacgagtgcgacatccccatcggcgccggcatctgcgccagctaccagacccagaccaagagccaccggcgggcccggagcgtggccagccagagcatcatcgcctacaccatgtccctgggcgccgagaacagcgtggcctacagcaacaacagcatcgccatccccaccaacttcaccatcagcgtgaccaccgagatcctgcccgtgagcatgaccaagaccagcgtggactgcaccatgtacatctgcggcgacagcaccgagtgcagcaacctgctgctgcagtacggcagcttctgcacccagctgaagcgggccctgaccggcatcgccgtggagcaggacaagaacacccaggaggtgttcgcccaggtgaagcagatctacaagaccccccccatcaagtacttcggcggcttcaacttcagccagatcctgcccgaccccagcaagcccagcaagcggagcttcatcgaggacctgctgttcaacaaggtgaccctggccgacgccggcttcatcaagcagtacggcgactgcctgggcgacatcgccgcccgggacctgatctgcgcccagaagttcaacggcctgaccgtgctgccccccctgctgaccgacgagatgatcgcccagtacaccagcgccctgctggccggcaccatcaccagcggctggaccttcggcgccggcgccgccctgcagatccccttcgccatgcagatggcctaccggttcaacggcatcggcgtgacccagaacgtgctgtacgagaaccagaagctgatcgccaaccagttcaacagcgccatcggcaagatccaggacagcctgagcagcaccgccagcgccctgggcaagctgcaggacgtggtgaaccacaacgcccaggccctgaacaccctggtgaagcagctgagcagcaagttcggcgccatcagcagcgtgctgaacgacatcctgagccggctggacccccccgaggccgaggtgcagatcgaccggctgatcaccggccggctgcagagcctgcagacctacgtgacccagcagctgatccgggccgccgagatccgggccagcgccaacctggccgccaccaagatgagcgagtgcgtgctgggccagagcaagcgggtggacttctgcggcaagggctaccacctgatgagcttcccccagagcgccccccacggcgtggtgttcctgcacgtgacctacgtgcccgcccaggagaagaacttcaccaccgcccccgccatctgccacgacggcaaggcccacttcccccgggagggcgtgttcgtgagcaacggcacccactggttcgtgacccagcggaacttctacgagccccagatcatcaccaccgacaacaccttcgtgagcggcaactgcgacgtggtgatcggcatcgtgaacaacaccgtgtacgaccccctgcagcccgagctggacagcttcaaggaggagctggacaagtacttcaagaaccacaccagccccgacgtggacctgggcgacatcagcggcatcaacgccagcgtggtgaacatccagaaggagatcgaccggctgaacgaggtggccaagaacctgaacgagagcctgatcgacctgcaggagctgggcaagtacgagcagtacatcaagtggccctggtacatctggctgggcttcatcgccggcctgatcgccatcgtgatggtgaccatcatgctgtgctgcatgaccagctgctgcagctgcctgaagggctgctgcagctgcggcagctgctgcaagttcgacgaggacgacagcgagcccgtgctgaagggcgtgaagctgcactacacctgatgactcgagctggtactgcatgcacgcaatgctagctgcccctttcccgtcctgggtaccccgagtctcccccgacctcgggtcccaggtatgctcccacctccacctgccccactcaccacctctgctagttccagacacctcccaagcacgcagcaatgcagctcaaaacgcttagcctagccacacccccacgggaaacagcagtgattaacctttagcaataaacgaaagtttaactaagctatactaaccccagggttggtcaatttcgtgccagccacaccctggagctagcaaaaaaaaaaaaaaaaaaaaaaaaaaaaaagcatatgactaaaaaaaaaaaaaaaaaaaaaaaaaaaaaaaaaaaaaaaaaaaaaaaaaaaaaaaaaaaaaaaaaaaaaa

SEQ ID NO: 22 - DNA, 4349 bp, synthetic construct
  source 1..4349: mol_type = other DNA
gggagacccaagctggctagcgtttaaacttaagcttggtaccgagctcggatccactagtccagtgtggtggaattcagaataaactagtattcttctggtccccacagactcagagagaacccgccaccatgttcgtttttttagttttattacctttagtgagcagccagtgcgtgaacctgatcacccggacccagagctacaccaacagcttcacccggggcgtgtactaccccgacaaggtgttccggagcagcgtgctgcacagcacccaggacctgttcctgcccttcttcagcaacgtgacctggttccacgccatccacgtgagcggcaccaacggcaccaagcggttcgacaaccccgccctgcccttcaacgacggcgtgtacttcgccagcaccgagaagagcaacatcatccggggctggatcttcggcaccaccctggacagcaagacccagagcctgctgatcgtgaacaacgccaccaacgtggtgatcaaggtgtgcgagttccagttctgcaacgaccccttcctggacgtgtaccagaagaacaacaagagctggatggagagcgagttccgggtgtacagcagcgccaacaactgcaccttcgagtacgtgagccagcccttcctgatggacctggagggcaaggagggcaacttcaagaacctgcgggagttcgtgttcaagaacatcgacggctacttcaagatctacagcaagcacacccccatcaacctggagcgggacctgccccagggcttcagcgccctggagcccctggtggacctgcccatcggcatcaacatcacccggttccagaccctgctggccctgcaccggagctacctgacccccgtggacagcagcagcggctggaccgccggcgccgccgcctactacgtgggctacctgcagccccggaccttcctgctgaagtacaacgagaacggcaccatcaccgacgccgtggactgcgccctggaccccctgagcgagaccaagtgcaccctgaagagcttcaccgtggagaagggcatctaccagaccagcaacttccgggtgcagcccaccgagagcatcgtgcggttccccaacatcaccaacctgtgccccttccacgaggtgttcaacgccaccaccttcgccagcgtgtacgcctggaaccggaagcggatcagcaactgcgtggccgactacagcgtgatctacaacttcgcccccttcttcgccttcaagtgctacggcgtgagccccaccaagctgaacgacctgtgcttcaccaacgtgtacgccgacagcttcgtgatccggggcaacgaggtgagccagatcgcccccggccagaccggcaacatcgccgactacaactacaagctgcccgacgacttcaccggctgcgtgatcgcctggaacagcaacaagctggacagcaagcccagcggcaactacaactacctgtaccggctgttccggaagagcaagctgaagcccttcgagcgggacatcagcaccgagatctaccaggccggcaacaagccctgcaacggcgtggccggccccaactgctacagccccctgcagagctacggcttccggcccacctacggcgtgggccaccagccctaccgggtggtggtgctgagcttcgagctgctgcacgcccccgccaccgtgtgcggccccaagaagagcaccaacctggtgaagaacaagtgcgtgaacttcaacttcaacggcctgaccggcaccggcgtgctgaccgagagcaacaagaagttcctgcccttccagcagttcggccgggacatcgccgacaccaccgacgccgtgcgggacccccagaccctggagatcctggacatcaccccctgcagcttcggcggcgtgagcgtgatcacccccggcaccaacaccagcaaccaggtggccgtgctgtaccagggcgtgaactgcaccgaggtgcccgtggccatccacgccgaccagctgacccccacctggcgggtgtacagcaccggcagcaacgtgttccagacccgggccggctgcctgatcggcgccgagtacgtgaacaacagctacgagtgcgacatccccatcggcgccggcatctgcgccagctaccagacccagaccaagagccaccggcgggcccggagcgtggccagccagagcatcatcgcctacaccatgagcctgggcgccgagaacagcgtggcctacagcaacaacagcatcgccatccccaccaacttcaccatctccgtgaccaccgagatcctgcccgtgagcatgaccaagaccagcgtggactgcaccatgtacatctgcggcgacagcaccgagtgcagcaacctgctgctgcagtacggcagcttctgcacccagctgaagcgggccctgaccggcatcgccgtggagcaggacaagaacacccaggaggtgttcgcccaggtgaagcagatctacaagaccccccccatcaagtacttcggcggcttcaacttcagccagatcctgcccgaccccagcaagcccagcaagcggagcttcatcgaggacctgctgttcaacaaggtgaccctggccgacgccggcttcatcaagcagtacggcgactgcctgggcgacatcgccgcccgggacctgatctgcgcccagaagttcaacggcctgaccgtgctgccccccctgctgaccgacgagatgatcgcccagtacaccagcgccctgctggccggcaccatcaccagcggctggaccttcggcgccggcgccgccctgcagatccccttcgccatgcagatggcctaccggttcaacggcatcggcgtgacccagaacgtgctgtacgagaaccagaagctgatcgccaaccagttcaacagcgccatcggcaagatccaggacagcctgagcagcaccgccagcgccctgggcaagctgcaggacgtggtgaaccacaacgcccaggccctgaacaccctggtgaagcagctgagcagcaagttcggcgccatcagcagcgtgctgaacgacatcctgagccggctggacccccccgaggccgaggtgcagatcgaccgcctgatcaccggccggctgcagagcctgcagacctacgtgacccagcagctgatccgggccgccgagatccgggccagcgccaacctggccgccaccaagatgagcgagtgcgtgctgggccagagcaagcgggtggacttctgcggcaagggctaccacctgatgagcttcccccagagcgccccccacggcgtggtgttcctgcacgtgacctacgtgcccgcccaggagaagaacttcaccaccgcccccgccatctgccacgacggcaaggcccacttcccccgggagggcgtgttcgtgagcaacggcacccactggttcgtgacccagcggaacttctacgagccccagatcatcaccaccgacaacaccttcgtgagcggcaactgcgacgtggtgatcggcatcgtgaacaacaccgtgtacgaccccctgcagcccgagctggacagcttcaaggaggagctggacaagtacttcaagaaccacaccagccccgacgtggacctgggcgacatcagcggcatcaacgccagcgtggtgaacatccagaaggagatcgaccggctgaacgaggtggccaagaacctgaacgagagcctgatcgacctgcaggagctgggcaagtacgagcagtacatcaagtggccctggtacatctggctgggcttcatcgccggcctgatcgccatcgtgatggtgaccatcatgctgtgctgcatgaccagctgctgcagctgcctgaagggctgctgcagctgcggcagctgctgcaagttcgacgaggacgacagcgagcccgtgctgaagggcgtgaagctgcactacacctgatgactcgagctggtactgcatgcacgcaatgctagctgcccctttcccgtcctgggtaccccgagtctcccccgacctcgggtcccaggtatgctcccacctccacctgccccactcaccacctctgctagttccagacacctcccaagcacgcagcaatgcagctcaaaacgcttagcctagccacacccccacgggaaacagcagtgattaacctttagcaataaacgaaagtttaactaagctatactaaccccagggttggtcaatttcgtgccagccacaccctggagctagcaaaaaaaaaaaaaaaaaaaaaaaaaaaaaagcatatgactaaaaaaaaaaaaaaaaaaaaaaaaaaaaaaaaaaaaaaaaaaaaaaaaaaaaaaaaaaaaaaaaaaaaaa

SEQ ID NO: 23 - DNA, 4349 bp, synthetic construct
  source 1..4349: mol_type = other DNA
gggagacccaagctggctagcgtttaaacttaagcttggtaccgagctcggatccactagtccagtgtggtggaattcagaataaactagtattcttctggtccccacagactcagagagaacccgccaccatgttcgtttttttagttttattacctttagtgagcagccagtgcgtgaacctgatcacccggacccagagctacaccaacagcttcacccggggcgtgtactaccccgacaaggtgttccggagcagcgtgctgcacagcacccaggacctgttcctgcccttcttcagcaacgtgacctggttccacgccatccacgtgagcggcaccaacggcaccaagcggttcgacaaccccgccctgcccttcaacgacggcgtgtacttcgccagcaccgagaagagcaacatcatccggggctggatcttcggcaccaccctggacagcaagacccagagcctgctgatcgtgaacaacgccaccaacgtggtgatcaaggtgtgcgagttccagttctgcaacgaccccttcctggacgtgtaccagaagaacaacaagagctggatggagagcgagttccgggtgtacagcagcgccaacaactgcaccttcgagtacgtgagccagcccttcctgatggacctggtgggcaaggagggcaacttcaagaacctgcgggagttcgtgttcaagaacatcgacggctacttcaagatctacagcaagcacacccccatcaacctggagcgggacctgccccagggcttcagcgccctggagcccctggtggacctgcccatcggcatcaacatcacccggttccagaccctgctggccctgcaccggagctacctgacccccgtggacagcagcagcggctggaccgccggcgccgccgcctactacgtgggctacctgcagccccggaccttcctgctgaagtacaacgagaacggcaccatcaccgacgccgtggactgcgccctggaccccctgagcgagaccaagtgcaccctgaagagcttcaccgtggagaagggcatctaccagaccagcaacttccgggtgcagcccaccgagagcatcgtgcggttccccaacatcaccaacctgtgccccttccacgaggtgttcaacgccaccaccttcgccagcgtgtacgcctggaaccggaagcggatcagcaactgcgtggccgactacagcgtgatctacaacttcgcccccttcttcgccttcaagtgctacggcgtgagccccaccaagctgaacgacctgtgcttcaccaacgtgtacgccgacagcttcgtgatccggggcaacgaggtgagccagatcgcccccggccagaccggcaacatcgccgactacaactacaagctgcccgacgacttcaccggctgcgtgatcgcctggaacagcaacaagctggacagcaagcccagcggcaactacaactacctgtaccggctgttccggaagagcaagctgaagcccttcgagcgggacatcagcaccgagatctaccaggccggcaaccggccctgcaacggcgtggccggccccaactgctacagccccctgcagagctacggcttccggcccacctacggcgtgggccaccagccctaccgggtggtggtgctgagcttcgagctgctgcacgcccccgccaccgtgtgcggccccaagaagagcaccaacctggtgaagaacaagtgcgtgaacttcaacttcaacggcctgaccggcaccggcgtgctgaccgagagcaacaagaagttcctgcccttccagcagttcggccgggacatcgccgacaccaccgacgccgtgcgggacccccagaccctggagatcctggacatcaccccctgcagcttcggcggcgtgagcgtgatcacccccggcaccaacaccagcaaccaggtggccgtgctgtaccagggcgtgaactgcaccgaggtgcccgtggccatccacgccgaccagctgacccccacctggcgggtgtacagcaccggcagcaacgtgttccagacccgggccggctgcctgatcggcgccgagtacgtgaacaacagctacgagtgcgacatccccatcggcgccggcatctgcgccagctaccagacccagaccaagagccaccggcgggcccggagcgtggccagccagagcatcatcgcctacaccatgagcctgggcgccgagaacagcgtggcctacagcaacaacagcatcgccatccccaccaacttcaccatctccgtgaccaccgagatcctgcccgtgagcatgaccaagaccagcgtggactgcaccatgtacatctgcggcgacagcaccgagtgcagcaacctgctgctgcagtacggcagcttctgcacccagctgaagcgggccctgaccggcatcgccgtggagcaggacaagaacacccaggaggtgttcgcccaggtgaagcagatctacaagaccccccccatcaagtacttcggcggcttcaacttcagccagatcctgcccgaccccagcaagcccagcaagcggagcttcatcgaggacctgctgttcaacaaggtgaccctggccgacgccggcttcatcaagcagtacggcgactgcctgggcgacatcgccgcccgggacctgatctgcgcccagaagttcaacggcctgaccgtgctgccccccctgctgaccgacgagatgatcgcccagtacaccagcgccctgctggccggcaccatcaccagcggctggaccttcggcgccggcgccgccctgcagatccccttcgccatgcagatggcctaccggttcaacggcatcggcgtgacccagaacgtgctgtacgagaaccagaagctgatcgccaaccagttcaacagcgccatcggcaagatccaggacagcctgagcagcaccgccagcgccctgggcaagctgcaggacgtggtgaaccacaacgcccaggccctgaacaccctggtgaagcagctgagcagcaagttcggcgccatcagcagcgtgctgaacgacatcctgagccggctggacccccccgaggccgaggtgcagatcgaccgcctgatcaccggccggctgcagagcctgcagacctacgtgacccagcagctgatccgggccgccgagatccgggccagcgccaacctggccgccaccaagatgagcgagtgcgtgctgggccagagcaagcgggtggacttctgcggcaagggctaccacctgatgagcttcccccagagcgccccccacggcgtggtgttcctgcacgtgacctacgtgcccgcccaggagaagaacttcaccaccgcccccgccatctgccacgacggcaaggcccacttcccccgggagggcgtgttcgtgagcaacggcacccactggttcgtgacccagcggaacttctacgagccccagatcatcaccaccgacaacaccttcgtgagcggcaactgcgacgtggtgatcggcatcgtgaacaacaccgtgtacgaccccctgcagcccgagctggacagcttcaaggaggagctggacaagtacttcaagaaccacaccagccccgacgtggacctgggcgacatcagcggcatcaacgccagcgtggtgaacatccagaaggagatcgaccggctgaacgaggtggccaagaacctgaacgagagcctgatcgacctgcaggagctgggcaagtacgagcagtacatcaagtggccctggtacatctggctgggcttcatcgccggcctgatcgccatcgtgatggtgaccatcatgctgtgctgcatgaccagctgctgcagctgcctgaagggctgctgcagctgcggcagctgctgcaagttcgacgaggacgacagcgagcccgtgctgaagggcgtgaagctgcactacacctgatgactcgagctggtactgcatgcacgcaatgctagctgcccctttcccgtcctgggtaccccgagtctcccccgacctcgggtcccaggtatgctcccacctccacctgccccactcaccacctctgctagttccagacacctcccaagcacgcagcaatgcagctcaaaacgcttagcctagccacacccccacgggaaacagcagtgattaacctttagcaataaacgaaagtttaactaagctatactaaccccagggttggtcaatttcgtgccagccacaccctggagctagcaaaaaaaaaaaaaaaaaaaaaaaaaaaaaagcatatgactaaaaaaaaaaaaaaaaaaaaaaaaaaaaaaaaaaaaaaaaaaaaaaaaaaaaaaaaaaaaaaaaaaaaaa

SEQ ID NO: 24 - DNA, 4539 bp, synthetic construct
  source 1..4539: mol_type = other DNA
gggagacccaagctggctagcgtttaaacttaagcttggtaccgagctcggatccactagtccagtgtggtggaattcagaataaactagtattcttctggtccccacagactcagagagaacccgccaccatgttcgtttttttagttttattacctttagtgagctcccagtgcgtgaacctgatcacccggacccagagctacaccaacagcttcacccggggcgtgtactaccccgacaaggtgttccggagcagcgtgctgcacagcacccaggacctgttcctgcccttcttcagcaacgtgacctggttccacgccatcagcggcaccaacggcaccaagcggttcgacaaccccgtgctgcccttcaacgacggcgtgtacttcgccagcaccgagaagagcaacatcatccggggctggatcttcggcaccaccctggacagcaagacccagagcctgctgatcgtgaacaacgccaccaacgtggtgatcaaggtgtgcgagttccagttctgcaacgaccccttcctggacgtgtactaccacaagaacaacaagagctggatggagagcgagttccgggtgtacagcagcgccaacaactgcaccttcgagtacgtgagccagcccttcctgatggacctggagggcaagcagggcaacttcaagaacctgcgggagttcgtgttcaagaacatcgacggctacttcaagatctacagcaagcacacccccatcaacctgggccgggacctgccccagggcttcagcgccctggagcccctggtggacctgcccatcggcatcaacatcacccggttccagaccctgctggccctgcaccggagctacctgacccccggcgacagcagcagcggctggaccgccggcgccgccgcctactacgtgggctacctgcagccccggaccttcctgctgaagtacaacgagaacggcaccatcaccgacgccgtggactgcgccctggaccccctgagcgagaccaagtgcaccctgaagagcttcaccgtggagaagggcatctaccagaccagcaacttccgggtgcagcccaccgagagcatcgtgcggttccccaacatcaccaacctgtgccccttcgacgaggtgttcaacgccacccggttcgccagcgtgtacgcctggaaccggaagcggatcagcaactgcgtggccgactacagcgtgctgtacaacttcgcccccttcttcgccttcaagtgctacggcgtgagccccaccaagctgaacgacctgtgcttcaccaacgtgtacgccgacagcttcgtgatccggggcaacgaggtgagccagatcgcccccggccagaccggcaacatcgccgactacaactacaagctgcccgacgacttcaccggctgcgtgatcgcctggaacagcaacaagctggacagcaaggtgggcggcaactacaactaccggtaccggctgttccggaagagcaacctgaagcccttcgagcgggacatcagcaccgagatctaccaggccggcaacaagccctgcaacggcgtggccggcgtgaactgctacttccccctgcagagctacggcttccggcccacctacggcgtgggccaccagccctaccgggtggtggtgctgagcttcgagctgctgcacgcccccgccaccgtgtgcggccccaagaagagcaccaacctggtgaagaacaagtgcgtgaacttcaacttcaacggcctgaccggcaccggcgtgctgaccgagagcaacaagaagttcctgcccttccagcagttcggccgggacatcgccgacaccaccgacgccgtgcgggacccccagaccctggagatcctggacatcaccccctgcagcttcggcggcgtgagcgtgatcacccccggcaccaacaccagcaaccaggtggccgtgctgtaccagggcgtgaactgcaccgaggtgcccgtggccatccacgccgaccagctgacccccacctggcgggtgtacagcaccggcagcaacgtgttccagacccgggccggctgcctgatcggcgccgagtacgtgaacaacagctacgagtgcgacatccccatcggcgccggcatctgcgcctcctaccagacccagaccaagagccaccggcgggcccggagcgtggccagccagagcatcatcgcctacaccatgagcctgggcgccgagaacagcgtggcctacagcaacaacagcatcgccatccccaccaacttcaccatcagcgtgaccaccgagatcctgcccgtgagcatgaccaagaccagcgtggactgcaccatgtacatctgcggcgacagcaccgagtgcagcaacctgctgctgcagtacggcagcttctgcacccagctgaagcgggccctgaccggcatcgccgtggagcaggacaagaacacccaggaggtgttcgcccaggtgaagcagatctacaagaccccccccatcaagtacttcggcggcttcaacttcagccagatcctgcccgaccccagcaagcccagcaagcggagcttcatcgaggacctgctgttcaacaaggtgaccctggccgacgccggcttcatcaagcagtacggcgactgcctgggcgacatcgccgcccgggacctgatctgcgcccagaagttcaacggcctgaccgtgctgccccccctgctgaccgacgagatgatcgcccagtacaccagcgccctgctggccggcaccatcaccagcggctggaccttcggcgccggcgccgccctgcagatccccttcgccatgcagatggcctaccggttcaacggcatcggcgtgacccagaacgtgctgtacgagaaccagaagctgatcgccaaccagttcaacagcgccatcggcaagatccaggacagcctgagcagcaccgccagcgccctgggcaagctgcaggacgtggtgaaccacaacgcccaggccctgaacaccctggtgaagcagctgagcagcaagttcggcgccatcagcagcgtgctgaacgacatcctgagccggctggacccccccgaggccgaggtgcagatcgaccggctgatcaccggccggctgcagagcctgcagacctacgtgacccagcagctgatccgggccgccgagatccgggccagcgccaacctggccgccaccaagatgagcgagtgcgtgctgggccagagcaagcgggtggacttctgcggcaagggctaccacctgatgagcttcccccagagcgccccccacggcgtggtgttcctgcacgtgacctacgtgcccgcccaggagaagaacttcaccaccgcccccgccatctgccacgacggcaaggcccacttcccccgggagggcgtgttcgtgagcaacggcacccactggttcgtgacccagcggaacttctacgagccccagatcatcaccaccgacaacaccttcgtgagcggcaactgcgacgtggtgatcggcatcgtgaacaacaccgtgtacgaccccctgcagcccgagctggacagcttcaaggaggagctggacaagtacttcaagaaccacaccagccccgacgtggacctgggcgacatcagcggcatcaacgccagcgtggtgaacatccagaaggagatcgaccggctgaacgaggtggccaagaacctgaacgagagcctgatcgacctgcaggagctgggcaagtacgagcagtacatcaagtggccctggtacatctggctgggcttcatcgccggcctgatcgccatcgtgatggtgaccatcatgctgtgctgcatgaccagctgctgcagctgcctgaagggctgctgcagctgcggcagctgctgcaagttcgacgaggacgacagcgagcccgtgctgaagggcgtgaagctgcactacacctgatgagctcgctttcttgctgtccaatttctattaaaggttcctttgttccctaagtccaactactaaactgggggatattatgaagggccttgagcatctggattctgcctaataaaaaacatttattttcattgcaattgccatgtgtatgtgggttcgcccacatactctgatgatccccaatcgtggcgtgtcggcctgcttcggcaggcactggcgccgggatcattcatggcaagctggagcctcggtggccatgcttcttgccccttgggcctccccccagcccctcctccccttcctgcacccgtacccccgtggtctttgaataaagtctgagtgggcggcactcgagctggtactgcatgcacgcaatgctagctgcccctttcccgtcctgggtaccccgagtctcccccgacctcgggtcccaggtatgctcccacctccacctgccccactcaccacctctgctagttccagacacctccaaaaaaaaaaaaaaaaaaaaaaaaaaaaaagcatatgactaaaaaaaaaaaaaaaaaaaaaaaaaaaaaaaaaaaaaaaaaaaaaaaaaaaaaaaaaaaaaaaaaaaaaa

SEQ ID NO: 25 - DNA, 4428 bp, synthetic construct
  source 1..4428: mol_type = other DNA
gggagacccaagctggctagcgtttaaacttaagcttggtaccgagctcggatccactagtccagtgtggtggaattcagaataaactagtattcttctggtccccacagactcagagagaacccgccaccatgttcgtttttttagttttattacctttagtgagctcccagtgcgtgaacctgatcacccggacccagagctacaccaacagcttcacccggggcgtgtactaccccgacaaggtgttccggagcagcgtgctgcacagcacccaggacctgttcctgcccttcttcagcaacgtgacctggttccacgccatcagcggcaccaacggcaccaagcggttcgacaaccccgtgctgcccttcaacgacggcgtgtacttcgccagcaccgagaagagcaacatcatccggggctggatcttcggcaccaccctggacagcaagacccagagcctgctgatcgtgaacaacgccaccaacgtggtgatcaaggtgtgcgagttccagttctgcaacgaccccttcctggacgtgtactaccacaagaacaacaagagctggatggagagcgagttccgggtgtacagcagcgccaacaactgcaccttcgagtacgtgagccagcccttcctgatggacctggagggcaagcagggcaacttcaagaacctgcgggagttcgtgttcaagaacatcgacggctacttcaagatctacagcaagcacacccccatcaacctgggccgggacctgccccagggcttcagcgccctggagcccctggtggacctgcccatcggcatcaacatcacccggttccagaccctgctggccctgcaccggagctacctgacccccggcgacagcagcagcggctggaccgccggcgccgccgcctactacgtgggctacctgcagccccggaccttcctgctgaagtacaacgagaacggcaccatcaccgacgccgtggactgcgccctggaccccctgagcgagaccaagtgcaccctgaagagcttcaccgtggagaagggcatctaccagaccagcaacttccgggtgcagcccaccgagagcatcgtgcggttccccaacatcaccaacctgtgccccttcgacgaggtgttcaacgccacccggttcgccagcgtgtacgcctggaaccggaagcggatcagcaactgcgtggccgactacagcgtgctgtacaacttcgcccccttcttcgccttcaagtgctacggcgtgagccccaccaagctgaacgacctgtgcttcaccaacgtgtacgccgacagcttcgtgatccggggcaacgaggtgagccagatcgcccccggccagaccggcaacatcgccgactacaactacaagctgcccgacgacttcaccggctgcgtgatcgcctggaacagcaacaagctggacagcaaggtgggcggcaactacaactaccggtaccggctgttccggaagagcaacctgaagcccttcgagcgggacatcagcaccgagatctaccaggccggcaacaagccctgcaacggcgtggccggcgtgaactgctacttccccctgcagagctacggcttccggcccacctacggcgtgggccaccagccctaccgggtggtggtgctgagcttcgagctgctgcacgcccccgccaccgtgtgcggccccaagaagagcaccaacctggtgaagaacaagtgcgtgaacttcaacttcaacggcctgaccggcaccggcgtgctgaccgagagcaacaagaagttcctgcccttccagcagttcggccgggacatcgccgacaccaccgacgccgtgcgggacccccagaccctggagatcctggacatcaccccctgcagcttcggcggcgtgagcgtgatcacccccggcaccaacaccagcaaccaggtggccgtgctgtaccagggcgtgaactgcaccgaggtgcccgtggccatccacgccgaccagctgacccccacctggcgggtgtacagcaccggcagcaacgtgttccagacccgggccggctgcctgatcggcgccgagtacgtgaacaacagctacgagtgcgacatccccatcggcgccggcatctgcgcctcctaccagacccagaccaagagccaccggcgggcccggagcgtggccagccagagcatcatcgcctacaccatgagcctgggcgccgagaacagcgtggcctacagcaacaacagcatcgccatccccaccaacttcaccatcagcgtgaccaccgagatcctgcccgtgagcatgaccaagaccagcgtggactgcaccatgtacatctgcggcgacagcaccgagtgcagcaacctgctgctgcagtacggcagcttctgcacccagctgaagcgggccctgaccggcatcgccgtggagcaggacaagaacacccaggaggtgttcgcccaggtgaagcagatctacaagaccccccccatcaagtacttcggcggcttcaacttcagccagatcctgcccgaccccagcaagcccagcaagcggagcttcatcgaggacctgctgttcaacaaggtgaccctggccgacgccggcttcatcaagcagtacggcgactgcctgggcgacatcgccgcccgggacctgatctgcgcccagaagttcaacggcctgaccgtgctgccccccctgctgaccgacgagatgatcgcccagtacaccagcgccctgctggccggcaccatcaccagcggctggaccttcggcgccggcgccgccctgcagatccccttcgccatgcagatggcctaccggttcaacggcatcggcgtgacccagaacgtgctgtacgagaaccagaagctgatcgccaaccagttcaacagcgccatcggcaagatccaggacagcctgagcagcaccgccagcgccctgggcaagctgcaggacgtggtgaaccacaacgcccaggccctgaacaccctggtgaagcagctgagcagcaagttcggcgccatcagcagcgtgctgaacgacatcctgagccggctggacccccccgaggccgaggtgcagatcgaccggctgatcaccggccggctgcagagcctgcagacctacgtgacccagcagctgatccgggccgccgagatccgggccagcgccaacctggccgccaccaagatgagcgagtgcgtgctgggccagagcaagcgggtggacttctgcggcaagggctaccacctgatgagcttcccccagagcgccccccacggcgtggtgttcctgcacgtgacctacgtgcccgcccaggagaagaacttcaccaccgcccccgccatctgccacgacggcaaggcccacttcccccgggagggcgtgttcgtgagcaacggcacccactggttcgtgacccagcggaacttctacgagccccagatcatcaccaccgacaacaccttcgtgagcggcaactgcgacgtggtgatcggcatcgtgaacaacaccgtgtacgaccccctgcagcccgagctggacagcttcaaggaggagctggacaagtacttcaagaaccacaccagccccgacgtggacctgggcgacatcagcggcatcaacgccagcgtggtgaacatccagaaggagatcgaccggctgaacgaggtggccaagaacctgaacgagagcctgatcgacctgcaggagctgggcaagtacgagcagtacatcaagtggccctggtacatctggctgggcttcatcgccggcctgatcgccatcgtgatggtgaccatcatgctgtgctgcatgaccagctgctgcagctgcctgaagggctgctgcagctgcggcagctgctgcaagttcgacgaggacgacagcgagcccgtgctgaagggcgtgaagctgcactacacctgatgagctcgctttcttgctgtccaatttctattaaaggttcctttgttccctaagtccaactactaaactgggggatattatgaagggccttgagcatctggattctgcctaataaaaaacatttattttcattgcaattgccatgtgtatgtgggttcgcccacatactctgatgatccccaatcgtggcgtgtcggcctgcttcggcaggcactggcgccgggatcattcatggcaactcgagctggtactgcatgcacgcaatgctagctgcccctttcccgtcctgggtaccccgagtctcccccgacctcgggtcccaggtatgctcccacctccacctgccccactcaccacctctgctagttccagacacctccaaaaaaaaaaaaaaaaaaaaaaaaaaaaaagcatatgactaaaaaaaaaaaaaaaaaaaaaaaaaaaaaaaaaaaaaaaaaaaaaaaaaaaaaaaaaaaaaaaaaaaaaa

SEQ ID NO: 26 - DNA, 4397 bp, synthetic construct
  source 1..4397: mol_type = other DNA
gggagacccaagctggctagcgtttaaacttaagcttggtaccgagctcggatccactagtccagtgtggtggaattcagaataaactagtattcttctggtccccacagactcagagagaacccgccaccatgttcgtttttttagttttattacctttagtgagctcccagtgcgtgaacctgatcacccggacccagagctacaccaacagcttcacccggggcgtgtactaccccgacaaggtgttccggagcagcgtgctgcacagcacccaggacctgttcctgcccttcttcagcaacgtgacctggttccacgccatcagcggcaccaacggcaccaagcggttcgacaaccccgtgctgcccttcaacgacggcgtgtacttcgccagcaccgagaagagcaacatcatccggggctggatcttcggcaccaccctggacagcaagacccagagcctgctgatcgtgaacaacgccaccaacgtggtgatcaaggtgtgcgagttccagttctgcaacgaccccttcctggacgtgtactaccacaagaacaacaagagctggatggagagcgagttccgggtgtacagcagcgccaacaactgcaccttcgagtacgtgagccagcccttcctgatggacctggagggcaagcagggcaacttcaagaacctgcgggagttcgtgttcaagaacatcgacggctacttcaagatctacagcaagcacacccccatcaacctgggccgggacctgccccagggcttcagcgccctggagcccctggtggacctgcccatcggcatcaacatcacccggttccagaccctgctggccctgcaccggagctacctgacccccggcgacagcagcagcggctggaccgccggcgccgccgcctactacgtgggctacctgcagccccggaccttcctgctgaagtacaacgagaacggcaccatcaccgacgccgtggactgcgccctggaccccctgagcgagaccaagtgcaccctgaagagcttcaccgtggagaagggcatctaccagaccagcaacttccgggtgcagcccaccgagagcatcgtgcggttccccaacatcaccaacctgtgccccttcgacgaggtgttcaacgccacccggttcgccagcgtgtacgcctggaaccggaagcggatcagcaactgcgtggccgactacagcgtgctgtacaacttcgcccccttcttcgccttcaagtgctacggcgtgagccccaccaagctgaacgacctgtgcttcaccaacgtgtacgccgacagcttcgtgatccggggcaacgaggtgagccagatcgcccccggccagaccggcaacatcgccgactacaactacaagctgcccgacgacttcaccggctgcgtgatcgcctggaacagcaacaagctggacagcaaggtgggcggcaactacaactaccggtaccggctgttccggaagagcaacctgaagcccttcgagcgggacatcagcaccgagatctaccaggccggcaacaagccctgcaacggcgtggccggcgtgaactgctacttccccctgcagagctacggcttccggcccacctacggcgtgggccaccagccctaccgggtggtggtgctgagcttcgagctgctgcacgcccccgccaccgtgtgcggccccaagaagagcaccaacctggtgaagaacaagtgcgtgaacttcaacttcaacggcctgaccggcaccggcgtgctgaccgagagcaacaagaagttcctgcccttccagcagttcggccgggacatcgccgacaccaccgacgccgtgcgggacccccagaccctggagatcctggacatcaccccctgcagcttcggcggcgtgagcgtgatcacccccggcaccaacaccagcaaccaggtggccgtgctgtaccagggcgtgaactgcaccgaggtgcccgtggccatccacgccgaccagctgacccccacctggcgggtgtacagcaccggcagcaacgtgttccagacccgggccggctgcctgatcggcgccgagtacgtgaacaacagctacgagtgcgacatccccatcggcgccggcatctgcgcctcctaccagacccagaccaagagccaccggcgggcccggagcgtggccagccagagcatcatcgcctacaccatgagcctgggcgccgagaacagcgtggcctacagcaacaacagcatcgccatccccaccaacttcaccatcagcgtgaccaccgagatcctgcccgtgagcatgaccaagaccagcgtggactgcaccatgtacatctgcggcgacagcaccgagtgcagcaacctgctgctgcagtacggcagcttctgcacccagctgaagcgggccctgaccggcatcgccgtggagcaggacaagaacacccaggaggtgttcgcccaggtgaagcagatctacaagaccccccccatcaagtacttcggcggcttcaacttcagccagatcctgcccgaccccagcaagcccagcaagcggagcttcatcgaggacctgctgttcaacaaggtgaccctggccgacgccggcttcatcaagcagtacggcgactgcctgggcgacatcgccgcccgggacctgatctgcgcccagaagttcaacggcctgaccgtgctgccccccctgctgaccgacgagatgatcgcccagtacaccagcgccctgctggccggcaccatcaccagcggctggaccttcggcgccggcgccgccctgcagatccccttcgccatgcagatggcctaccggttcaacggcatcggcgtgacccagaacgtgctgtacgagaaccagaagctgatcgccaaccagttcaacagcgccatcggcaagatccaggacagcctgagcagcaccgccagcgccctgggcaagctgcaggacgtggtgaaccacaacgcccaggccctgaacaccctggtgaagcagctgagcagcaagttcggcgccatcagcagcgtgctgaacgacatcctgagccggctggacccccccgaggccgaggtgcagatcgaccggctgatcaccggccggctgcagagcctgcagacctacgtgacccagcagctgatccgggccgccgagatccgggccagcgccaacctggccgccaccaagatgagcgagtgcgtgctgggccagagcaagcgggtggacttctgcggcaagggctaccacctgatgagcttcccccagagcgccccccacggcgtggtgttcctgcacgtgacctacgtgcccgcccaggagaagaacttcaccaccgcccccgccatctgccacgacggcaaggcccacttcccccgggagggcgtgttcgtgagcaacggcacccactggttcgtgacccagcggaacttctacgagccccagatcatcaccaccgacaacaccttcgtgagcggcaactgcgacgtggtgatcggcatcgtgaacaacaccgtgtacgaccccctgcagcccgagctggacagcttcaaggaggagctggacaagtacttcaagaaccacaccagccccgacgtggacctgggcgacatcagcggcatcaacgccagcgtggtgaacatccagaaggagatcgaccggctgaacgaggtggccaagaacctgaacgagagcctgatcgacctgcaggagctgggcaagtacgagcagtacatcaagtggccctggtacatctggctgggcttcatcgccggcctgatcgccatcgtgatggtgaccatcatgctgtgctgcatgaccagctgctgcagctgcctgaagggctgctgcagctgcggcagctgctgcaagttcgacgaggacgacagcgagcccgtgctgaagggcgtgaagctgcactacacctgatgagctcgctttcttgctgtccaatttctattaaaggttcctttgttccctaagtccaactactaaactgggggatattatgaagggccttgagcatctggattctgcctaataaaaaacatttattttcattgcaattgccatgtgtatgtgggttcgcccacatactctgatgatccccaatcgtggcgtgtcggcctgcttcggcaggcactggcgccgggatcattcatggcaagctggagcctcggtggccatgcttcttgccccttgggcctccccccagcccctcctccccttcctgcacccgtacccccgtggtctttgaataaagtctgagtgggcggcaaaaaaaaaaaaaaaaaaaaaaaaaaaaaaagcatatgactaaaaaaaaaaaaaaaaaaaaaaaaaaaaaaaaaaaaaaaaaaaaaaaaaaaaaaaaaaaaaaaaaaaaaa

SEQ ID NO: 27 - RNA, 1653 nt, synthetic construct
  source 1..1653: mol_type = other RNA
atggaagacgccaaaaacataaagaaaggcccggcgccattctatccgctggaagatggaaccgctggagagcaactgcataaggctatgaagagatacgccctggttcctggaacaattgcttttacagatgcacatatcgaggtggacatcacttacgctgagtacttcgaaatgtccgttcggttggcagaagctatgaaacgatatgggctgaatacaaatcacagaatcgtcgtatgcagtgaaaactctcttcaattctttatgccggtgttgggcgcgttatttatcggagttgcagttgcgcccgcgaacgacatttataatgaacgtgaattgctcaacagtatgggcatttcgcagcctaccgtggtgttcgtttccaaaaaggggttgcaaaaaattttgaacgtgcaaaaaaagctcccaatcatccaaaaaattattatcatggattctaaaacggattaccagggatttcagtcgatgtacacgttcgtcacatctcatctacctcccggttttaatgaatacgattttgtgccagagtccttcgatagggacaagacaattgcactgatcatgaactcctctggatctactggtctgcctaaaggtgtcgctctgcctcatagaactgcctgcgtgagattctcgcatgccagagatcctatttttggcaatcaaatcattccggatactgcgattttaagtgttgttccattccatcacggttttggaatgtttactacactcggatatttgatatgtggatttcgagtcgtcttaatgtatagatttgaagaagagctgtttctgaggagccttcaggattacaagattcaaagtgcgctgctggtgccaaccctattctccttcttcgccaaaagcactctgattgacaaatacgatttatctaatttacacgaaattgcttctggtggcgctcccctctctaaggaagtcggggaagcggttgccaagaggttccatctgccaggtatcaggcaaggatatgggctcactgagactacatcagctattctgattacacccgagggggatgataaaccgggcgcggtcggtaaagttgttccattttttgaagcgaaggttgtggatctggataccgggaaaacgctgggcgttaatcaaagaggcgaactgtgtgtgagaggtcctatgattatgtccggttatgtaaacaatccggaagcgaccaacgccttgattgacaaggatggatggctacattctggagacatagcttactgggacgaagacgaacacttcttcatcgttgaccgcctgaagtctctgattaagtacaaaggctatcaggtggctcccgctgaattggaatccatcttgctccaacaccccaacatcttcgacgcaggtgtcgcaggtcttcccgacgatgacgccggtgaacttcccgccgccgttgttgttttggagcacggaaagacgatgacggaaaaagagatcgtggattacgtcgccagtcaagtaacaaccgcgaaaaagttgcgcggaggagttgtgtttgtggacgaagtaccgaaaggtcttaccggaaaactcgacgcaagaaaaatcagagagatcctcataaaggccaagaagggcggaaagatcgccgtgtaa

SEQ ID NO: 28 - DNA, 21 bp, synthetic construct
  source 1..21: mol_type = other DNA
  modified_base 7: mod_base = um
  modified_base 17: mod_base = um
  misc_feature 1..19: note = RNA
atggaatactcttggttactt

SEQ ID NO: 29 - DNA, 21 bp, synthetic construct
  source 1..21: mol_type = other DNA
  modified_base 2: mod_base = um
  modified_base 5..6: mod_base = cm
  modified_base 12: mod_base = um
  modified_base 14..15: mod_base = um
  modified_base 16..17: mod_base = cm
  modified_base 19: mod_base = um
  misc_feature 1..19: note = RNA
gtaaccaagagtattccattt

SEQ ID NO: 30 - DNA, 20 bp, synthetic construct
  source 1..20: mol_type = other DNA
agcgtgctctataactcggc

SEQ ID NO: 31 - DNA, 20 bp, synthetic construct
  source 1..20: mol_type = other DNA
tcggacctcatcgcctctaa

SEQ ID NO: 32 - DNA, 20 bp, synthetic construct
  source 1..20: mol_type = other DNA
acggcgtgagccccacaaag